European Patent Specification EP 4 037 708 B1, published September 18, 2024. Title: HBV VACCINES AND METHODS TREATING HBV. Applicant: GILEAD SCIENCES, INC. The sequence listing filed with the application follows.

SEQUENCE LISTING (102 sequences)

SEQ ID NO: 1 - protein, 226 aa, Hepatitis B virus
MENITSGFLGPLLVLQAGFFLLTRILTIPQSLDSWWTSLNFLGGTPVCLGQNSQSPTSNHSPTSCPPICPGYRWMCLRRFIIFLFILLLCLIFLLVLLDYQGMLPVCPLIPGSTTTSTGPCKTCTTPAQGNSMFPSCCCTKPTDGNCTCIPIPSSWAFAKYLWEWASVRFSWLSLLVPFVQWFVGLSPTVWLSVIWMMWYWGPSLYNILSPFIPLLPIFFCLWVYI

SEQ ID NO: 2 - protein, 226 aa, Hepatitis B virus
MESTTSGFLGPLLVLQAGFFLLTRILTIPQSLDSWWTSLNFLGGAPTCPGQNLQSPTSNHSPTSCPPICPGYRWMCLRRFIIFLFILLLCLIFLLVLLDYQGMLPVCPLIPGSSTTSTGPCRTCTTPAQGTSMFPSCCCTKPTDGNCTCIPIPSSWAFAKYLWEWASVRFSWLSLLVPFVQWFVGLSPTVWLSVIWMMWYWGPSLYNILSPFMPLLPIFFCLWVYI

SEQ ID NO: 3 - protein, 226 aa, Hepatitis B virus
MESTTSGFLGPLLVLQAGFFLLTRILTIPQSLDSWWTSLNFLGGAPTCPGQNSQSPTSNHSPTSCPPICPGYRWMCLRRFIIFLCILLLCLIFLLVLLDYQGMLPVCPLIPGSSTTSTGPCKTCTTPAQGTSMFPSCCCTKPTDGNCTCIPIPSSWAFARFLWEWASVRFSWLSLLVPFVQWFVGLSPTVWLSVIWMMWYWGPSLYNILSPFLPLLPIFFCLWVYI

SEQ ID NO: 4 - protein, 226 aa, Hepatitis B virus
MENITSGFLGPLLVLQAGFFLLTRILTIPQSLDSWWTSLNFLGGTTVCLGQNSQSPTSNHSPTSCPPICPGYRWMCLRRFIIFLFILLLCLIFLLVLLDYQGMLPVCPLIPGSSTTSTGPCRTCTTPAQGTSMYPSCCCTKPSDGNCTCIPIPSSWAFGKFLWEWASARFSWLSLLVPFVQWFVGLSPTVWLSVIWMMWYWGPSLYSILSPFLPLLPIFFCLWVYI

SEQ ID NO: 5 - protein, 755 aa, Artificial Sequence
  source: /note="Description of Artificial Sequence: Synthetic polypeptide"
MPLSYQHFRKLLLLDDETEAGPLEEELPRLADEDLNRRVAEDLNLGNLNVSIPWTHKVGNFTGLYSSTVPIFNPEWQTPSFPKIHLHEDIANRCQQFVGPLTVNEKRRLRLIMPARFYPNSTKYLPLDKGIKPYYPDHVVNHYFQTRHYLHTLWKAGILYKRETTRSASFCGSPYSWEQELHHGRLVIKTSQRHGDEPFCSQPSGILSRSSVGPEFHSFPPSSARSQSQGPVFSCWWLQFRNTQPCSKYCLSHLVNLLEDWGPCDEHGEHHIRIPRTPARVTGGVFLVDKNPHNTAESRLVVDFSQFSRGITRVSWPKFAVPNLQSLTNLLSSNLSWLSLDVSAAFYHIPLHPAAMPHLLVGSSGLSRYVARLSSNSRIHNNQHGTLQNLHDSCSRQLYVSLMLLYKTYGRKLHLYSHPIILGFRKIPMGVGLSPFLLAQFTSAICSVVRRAFPHCLAFSYMHDVVLGAKSVQHLESLYTAVTNFLLSLGIHLNPNKTKRWGYSLNFMGYVIGSWGTLPQDHIVQKIKHCFRKLPINRPIDWKVCQRIVGLLGFAAPFTQCGYPALMPLYACIQAKQAFTFSPTYKAFLSKQYLNLYPVARQRPGLCQVFADATPTGWGLAIGHQRMRGTFVAPLPIHTAHLLAACFARSRSGAKLIGTDNSVVLSRKYTSFPWLLGCTANWILRGTSFVYVPSALNPADDPSRGRLGLYRPLLRLPYRPTTGRTSLYAVSPSVPSHLPVRVHFASPLHVAWRPP

SEQ ID NO: 6 - protein, 749 aa, Artificial Sequence
  source: /note="Description of Artificial Sequence: Synthetic polypeptide"
MPLSYQHFRKLLLLDDEAGPLEEELPRLADEGLNRRVAEDLNLGNLNVSIPWTHKVGNFTGLYSSTVPVFNPEWQTPSFPHIHLQEDIINRCQQYVGPLTVNEKRRLKLIMPARFYPNLTKYLPLDKGIKPYYPEHVVNHYFQTRHYLHTLWKAGILYKRESTRSASFCGSPYSWEQDLQHGRLVFQTSKRHGDKSFCPQSPGILPRSELHHFPPSSSRSQSQGPVLSCWWLQFRNSEPCSEYCLCHIVNLIEDWGPCTEHGEHRIRTPRTPARVTGGVFLVDKNPHNTTESRLVVDFSQFSRGNTRVSWPKFAVPNLQSLTNLLSSNLSWLSLDVSAAFYHLPLHPAAMPHLLVGSSGLSRYVARLSSNSRIINNQHRTMQNLHDSCSRNLYVSLMLLYKTYGRKLHLYSHPIILGFRKIPMGVGLSPFLLAQFTSAICSVVRRAFPHCLAFSYMHDVVLGAKSVQHLESLYAAVTNFLLSLGIHLNPHKTKRWGYSLNFMGYVIGSWGTLPQEHIVQKIKMCFRKLPVNRPIDWKVCQRIVGLLGFAAPFTQCGYPALMPLYACIQAKQAFTFSPTYKAFLSKQYLHLYPVARQRPGLCQVFADATPTGWGLAIGHQRMRGAFVSPLPIHTAHLLAACFARSRSGAKLIGTDNSVVLSRKYTSFPWLLGCAANWILRGTSFVYVPSALNPADDPSRGRLGLYRPLLRLLYRPTTGRTSLYADSPSVPSHLPDRVHFASPLHVAWRPP

SEQ ID NO: 7 - protein, 753 aa, Artificial Sequence
  source: /note="Description of Artificial Sequence: Synthetic polypeptide"
MPLSYQHFRKLLLLDDEAGPLEEELPRLADEDLNRRVAEDLNLGNLNVSIPWTHKVGNFTGLYSSTVPVFNPEWQTPSFPHIHLQEDIINRCQQYVGPLTVNEKRRLKLIMPARFYPNLTKYLPLDKGIKPYYPEHTVNHYFKTRHYLHTLWKAGILYKRETTRSASFCGSPYSWEQELQHGRLVFQTSTRHGDESFCSQSSGILSRSPVGPELHNFPPSSARSQSEGPLLSCWWLQFRNSKPCSDYCLSHIVNLLEDWGPCTEHGEHNIRIPRTPARVTGGVFLVDKNPHNTTESRLVVDFSQFSRGSTHVSWPKFAVPNLQSLTNLLSSNLSWLSLDVSAAFYHLPLHPAAMPHLLVGSSGLSRYVARLSSTSRNINYQHGAMQDLHDSCSRNLYVSLLLLYKTFGRKLHLYSHPIILGFRKIPMGVGLSPFLLAQFTSAICSVVRRAFPHCLAFSYMHDVVLGAKSVQHLESLFTAVTNFLLSLGIHLNPNKTKRWGYSLNFMGYVIGSWGTLPQEHIVLKIKQCFRKLPVNRPIDWKVCQRIVGLLGFAAPFTQCGYPALMPLYACIQAKQAFTFSPTYKAFLCKQYLNLYPVARQRSGLCQVFADATPTGWGLAVGHQRMRGTFVSPLPIHTAHLLAACFARSRSGAKLIGTDNSVVLSRKYTSFPWLLGCAANWILRGTSFVYVPSALNPADDPSRGRLGLYRPLLRLPFRPTTGRTSLYAVSPSVPSHLPVRVHFASPLHVAWRPP

SEQ ID NO: 8 - protein, 742 aa, Artificial Sequence
  source: /note="Description of Artificial Sequence: Synthetic polypeptide"
MPLSYQHFRRLLLLDDEAGPLEEELPRLADEGLNRRVAEDLNLGNLNVSIPWTHKVGNFTGLYSSTVPVFNPHWKTPSFPNIHLHQDIIKKCEQFVGPLTVNEKRRLQLIMPARFYPNVTKYLPLDKGIKPYYPEHLVNHYFQTRHYLHTLWKAGILYKRETTHSASFCGSPYSWEQELQHGAESFHQQSSGILSRPPVGSELHNLPPNSARSQSERPVFPCWWLQFRNSKPCSDYCLSHIVNLLEDWGPCAEHGEHHIRIPRTPARVTGGVFLVDKNPHNTAESRLVVDFSQFSRGNYRVSWPKFAVPNLQSLTNLLSSNLSWLSLDVSAAFYHLPLHPAAMPHLLVGSSGLSRYVARLSSNSRIFNYQHGTMQNLHDSCSRNLYVSLMLLYQTFGRKLHLYSHPIILGFRKIPMGVGLSPFLLAQFTSAICSVVRRAFPHCLAFSYMHDVVLGAKSVQHLESLFTAVTNFLLSLGIHLNPNKTKRWGYSLHFMGYVIGCYGSLPQDHIIQKIKECFRKLPVNRPIDWKVCQRIVGLLGFAAPFTQCGYPALMPLYACIQSKQAFTFSPTYKAFLCKQYLNLYPVARQRPGLCQVFADATPTGWGLVMGHQRMRGTFKAPLPIHTAHLLAACFARSRSGANILGTDNSVVLSRKYTSFPWLLGCAANWILRGTSFVYVPSALNPADDPSRGRLGLYRPLLRLPFRPTTGRTSLYADSPSVPSHLPDRVHFASPLHVAWRPP

SEQ ID NO: 9 - protein, 705 aa, Artificial Sequence
  source: /note="Description of Artificial Sequence: Synthetic polypeptide"
MPLSYQHFRKLLLLDDETEAGPLEEELPRLADEDLNRRVAEDLNLGNLNVSIPWTHKVGNFTGLYSSTVPIFNPEWQTPSFPKIHLHEDIANRCQQFVGPLTVNEKRRLRLIMPARFYPNSTKYLPLDKGIKPYYPDHVVNHYFQTRHYLHTLWKAGILYKRETTRSASFCGSPYSWEQELHHGCWWLQFRNTQPCSKYCLSHLVNLLEDWGPCDEHGEHHIRIPRTPARVTGGVFLVDKNPHNTAESRLVVDFSQFSRGITRVSWPKFAVPNLQSLTNLLSSNLSWLSLDVSAAFYHIPLHPAAMPHLLVGSSGLSRYVARLSSNSRIHNNQHGTLQNLHDSCSRQLYVSLMLLYKTYGRKLHLYSHPIILGFRKIPMGVGLSPFLLAQFTSAICSVVRRAFPHCLAFSYMHDVVLGAKSVQHLESLYTAVTNFLLSLGIHLNPNKTKRWGYSLNFMGYVIGSWGTLPQDHIVQKIKHCFRKLPINRPIDWKVCQRIVGLLGFAAPFTQCGYPALMPLYACIQAKQAFTFSPTYKAFLSKQYLNLYPVARQRPGLCQVFADATPTGWGLAIGHQRMRGTFVAPLPIHTAHLLAACFARSRSGAKLIGTDNSVVLSRKYTSFPWLLGCTANWILRGTSFVYVPSALNPADDPSRGRLGLYRPLLRLPYRPTTGRTSLYAVSPSVPSHLPVRVHFASPLHVAWRPP

SEQ ID NO: 10 - protein, 703 aa, Artificial Sequence
  source: /note="Description of Artificial Sequence: Synthetic polypeptide"
MPLSYQHFRKLLLLDDEAGPLEEELPRLADEGLNRRVAEDLNLGNLNVSIPWTHKVGNFTGLYSSTVPVFNPEWQTPSFPHIHLQEDIINRCQQYVGPLTVNEKRRLKLIMPARFYPNLTKYLPLDKGIKPYYPEHVVNHYFQTRHYLHTLWKAGILYKRESTRSASFCGSPYSWEQDLQHGCWWLQFRNSEPCSEYCLCHIVNLIEDWGPCTEHGEHRIRTPRTPARVTGGVFLVDKNPHNTTESRLVVDFSQFSRGNTRVSWPKFAVPNLQSLTNLLSSNLSWLSLDVSAAFYHLPLHPAAMPHLLVGSSGLSRYVARLSSNSRIINNQHRTMQNLHDSCSRNLYVSLMLLYKTYGRKLHLYSHPIILGFRKIPMGVGLSPFLLAQFTSAICSVVRRAFPHCLAFSYMHDVVLGAKSVQHLESLYAAVTNFLLSLGIHLNPHKTKRWGYSLNFMGYVIGSWGTLPQEHIVQKIKMCFRKLPVNRPIDWKVCQRIVGLLGFAAPFTQCGYPALMPLYACIQAKQAFTFSPTYKAFLSKQYLHLYPVARQRPGLCQVFADATPTGWGLAIGHQRMRGAFVSPLPIHTAHLLAACFARSRSGAKLIGTDNSVVLSRKYTSFPWLLGCAANWILRGTSFVYVPSALNPADDPSRGRLGLYRPLLRLLYRPTTGRTSLYADSPSVPSHLPDRVHFASPLHVAWRPP

SEQ ID NO: 11 - protein, 703 aa, Artificial Sequence
  source: /note="Description of Artificial Sequence: Synthetic polypeptide"
MPLSYQHFRKLLLLDDEAGPLEEELPRLADEDLNRRVAEDLNLGNLNVSIPWTHKVGNFTGLYSSTVPVFNPEWQTPSFPHIHLQEDIINRCQQYVGPLTVNEKRRLKLIMPARFYPNLTKYLPLDKGIKPYYPEHTVNHYFKTRHYLHTLWKAGILYKRETTRSASFCGSPYSWEQELQHGCWWLQFRNSKPCSDYCLSHIVNLLEDWGPCTEHGEHNIRIPRTPARVTGGVFLVDKNPHNTTESRLVVDFSQFSRGSTHVSWPKFAVPNLQSLTNLLSSNLSWLSLDVSAAFYHLPLHPAAMPHLLVGSSGLSRYVARLSSTSRNINYQHGAMQDLHDSCSRNLYVSLLLLYKTFGRKLHLYSHPIILGFRKIPMGVGLSPFLLAQFTSAICSVVRRAFPHCLAFSYMHDVVLGAKSVQHLESLFTAVTNFLLSLGIHLNPNKTKRWGYSLNFMGYVIGSWGTLPQEHIVLKIKQCFRKLPVNRPIDWKVCQRIVGLLGFAAPFTQCGYPALMPLYACIQAKQAFTFSPTYKAFLCKQYLNLYPVARQRSGLCQVFADATPTGWGLAVGHQRMRGTFVSPLPIHTAHLLAACFARSRSGAKLIGTDNSVVLSRKYTSFPWLLGCAANWILRGTSFVYVPSALNPADDPSRGRLGLYRPLLRLPFRPTTGRTSLYAVSPSVPSHLPVRVHFASPLHVAWRPP

SEQ ID NO: 12 - protein, 703 aa, Artificial Sequence
  source: /note="Description of Artificial Sequence: Synthetic polypeptide"
MPLSYQHFRRLLLLDDEAGPLEEELPRLADEGLNRRVAEDLNLGNLNVSIPWTHKVGNFTGLYSSTVPVFNPHWKTPSFPNIHLHQDIIKKCEQFVGPLTVNEKRRLQLIMPARFYPNVTKYLPLDKGIKPYYPEHLVNHYFQTRHYLHTLWKAGILYKRETTHSASFCGSPYSWEQELQHGCWWLQFRNSKPCSDYCLSHIVNLLEDWGPCAEHGEHHIRIPRTPARVTGGVFLVDKNPHNTAESRLVVDFSQFSRGNYRVSWPKFAVPNLQSLTNLLSSNLSWLSLDVSAAFYHLPLHPAAMPHLLVGSSGLSRYVARLSSNSRIFNYQHGTMQNLHDSCSRNLYVSLMLLYQTFGRKLHLYSHPIILGFRKIPMGVGLSPFLLAQFTSAICSVVRRAFPHCLAFSYMHDVVLGAKSVQHLESLFTAVTNFLLSLGIHLNPNKTKRWGYSLHFMGYVIGCYGSLPQDHIIQKIKECFRKLPVNRPIDWKVCQRIVGLLGFAAPFTQCGYPALMPLYACIQSKQAFTFSPTYKAFLCKQYLNLYPVARQRPGLCQVFADATPTGWGLVMGHQRMRGTFKAPLPIHTAHLLAACFARSRSGANILGTDNSVVLSRKYTSFPWLLGCAANWILRGTSFVYVPSALNPADDPSRGRLGLYRPLLRLPFRPTTGRTSLYADSPSVPSHLPDRVHFASPLHVAWRPP

SEQ ID NO: 13 - protein, 534 aa, Artificial Sequence
  source: /note="Description of Artificial Sequence: Synthetic polypeptide"
MSSRSQSQGPVLSCWWLQFRNSEPCSEYCLCHIVNLIEDWGPCTEHGEHRIRTPRTPARVTGGVFLVDKNPHNTTESRLVVDFSQFSRGNTRVSWPKFAVPNLQSLTNLLSSNLSWLSLDVSAAFYHLPLHPAAMPHLLVGSSGLSRYVARLSSNSRIINNQHRTMQNLHDSCSRNLYVSLMLLYKTYGRKLHLYSHPIILGFRKIPMGVGLSPFLLAQFTSAICSVVRRAFPHCLAFSYMHDVVLGAKSVQHLESLYAAVTNFLLSLGIHLNPHKTKRWGYSLNFMGYVIGSWGTLPQEHIVQKIKMCFRKLPVNRPIDWKVCQRIVGLLGFAAPFTQCGYPALMPLYACIQAKQAFTFSPTYKAFLSKQYLHLYPVARQRPGLCQVFADATPTGWGLAIGHQRMRGAFVSPLPIHTAHLLAACFARSRSGAKLIGTDNSVVLSRKYTSFPWLLGCAANWILRGTSFVYVPSALNPADDPSRGRLGLYRPLLRLLYRPTTGRTSLYADSPSVPSHLPDRVHFASPLHVAWRPP

SEQ ID NO: 14 - protein, 534 aa, Artificial Sequence
  source: /note="Description of Artificial Sequence: Synthetic polypeptide"
MSARSQSERPVFPCWWLQFRNSKPCSDYCLSHIVNLLEDWGPCAEHGEHHIRIPRTPARVTGGVFLVDKNPHNTAESRLVVDFSQFSRGNYRVSWPKFAVPNLQSLTNLLSSNLSWLSLDVSAAFYHLPLHPAAMPHLLVGSSGLSRYVARLSSNSRIFNYQHGTMQNLHDSCSRNLYVSLMLLYQTFGRKLHLYSHPIILGFRKIPMGVGLSPFLLAQFTSAICSVVRRAFPHCLAFSYMHDVVLGAKSVQHLESLFTAVTNFLLSLGIHLNPNKTKRWGYSLHFMGYVIGCYGSLPQDHIIQKIKECFRKLPVNRPIDWKVCQRIVGLLGFAAPFTQCGYPALMPLYACIQSKQAFTFSPTYKAFLCKQYLNLYPVARQRPGLCQVFADATPTGWGLVMGHQRMRGTFKAPLPIHTAHLLAACFARSRSGANILGTDNSVVLSRKYTSFPWLLGCAANWILRGTSFVYVPSALNPADDPSRGRLGLYRPLLRLPFRPTTGRTSLYADSPSVPSHLPDRVHFASPLHVAWRPP

SEQ ID NO: 15 - protein, 1030 aa, Artificial Sequence
  source: /note="Description of Artificial Sequence: Synthetic polypeptide"
MDIDPYKEFGASVELLSFLPSDFFPSVRDLLDTASALYREALESPEHCSPHHTALRQAILCWGELMTLATWVGNNLEDPASRDLVVNYVNTNMGLKIRQLLWFHISCLTFGRETVLEYLVSFGVWIRTPPAYRPPNAPILSTLPETTVVRRRDRGRSPRRRTPSPRRRRSQSPRRRRSQSRESQCMPLSYQHFRKLLLLDDETEAGPLEEELPRLADEDLNRRVAEDLNLGNLNVSIPWTHKVGNFTGLYSSTVPIFNPEWQTPSFPKIHLHEDIANRCQQFVGPLTVNEKRRLRLIMPARFYPNSTKYLPLDKGIKPYYPDHVVNHYFQTRHYLHTLWKAGILYKRETTRSASFCGSPYSWEQELHHGRLVIKTSQRHGDEPFCSQPSGILSRSSVGPCIRSQFKQSRLGLQPHQGPLATSQSGRSGSIRARVHSPTRRCFGVEPSGSGHIGHSASSSSSCLHQSAVRKAAYSHLSTSKRQSSSGHAVEFHSFPPSSARSQSQGPVFSCWWLQFRNTQPCSKYCLSHLVNLLEDWGPCDEHGEHHIRIPRTPARVTGGVFLVDKNPHNTAESRLVVDFSQFSRGITRVSWPKFAVPNLQSLTNLLSSNLSWLSLDVSAAFYHIPLHPAAMPHLLVGSSGLSRYVARLSSNSRIHNNQHGTLQNLHDSCSRQLYVSLMLLYKTYGRKLHLYSHPIILGFRKIPMGVGLSPFLLAQFTSAICSVVRRAFPHCLAFSYMHDVVLGAKSVQHLESLYTAVTNFLLSLGIHLNPNKTKRWGYSLNFMGYVIGSWGTLPQDHIVQKIKHCFRKLPINRPIDWKVCQRIVGLLGFAAPFTQCGYPALMPLYACIQAKQAFTFSPTYKAFLSKQYLNLYPVARQRPGLCQVFADATPTGWGLAIGHQRMRGTFVAPLPIHTAHLLAACFARSRSGAKLIGTDNSVVLSRKYTSFPWLLGCTANWILRGTSFVYVPSALNPADDPSRGRLGLYRPLLRLPYRPTTGRTSLYAVSPSVPSHLPVRVHFASPLHVAWRPP

SEQ ID NO: 16 - protein, 1026 aa, Artificial Sequence
  source: /note="Description of Artificial Sequence: Synthetic polypeptide"
MDIDPYKEFGASVELLSFLPSDFFPSVRDLLDTASALYREALESPEHCSPHHTALRQAILCWGELMNLATWVGSNLEDPASRELVVSYVNVNMGLKIRQLLWFHISCLTFGRETVLEYLVSFGVWIRTPPAYRPPNAPILSTLPETTVVRRRGRSPRRRTPSPRRRRSQSPRRRRSQSRESQCMPLSYQHFRKLLLLDDEAGPLEEELPRLADEGLNRRVAEDLNLGNLNVSIPWTHKVGNFTGLYSSTVPVFNPEWQTPSFPHIHLQEDIINRCQQYVGPLTVNEKRRLKLIMPARFYPNLTKYLPLDKGIKPYYPEHVVNHYFQTRHYLHTLWKAGILYKRESTRSASFCGSPYSWEQDLQHGRLVFQTSKRHGDKSFCPQSPGILPRSSVGPCIQNQLRKSRLGPQPAQGQLAGRQQGGSGSIRARVHPSPWGTVGVEPSGSGHIHNCASNSSSCLHQSAVRKAAYSHISTSKGHSSSGHAVELHHFPPSSSRSQSQGPVLSCWWLQFRNSEPCSEYCLCHIVNLIEDWGPCTEHGEHRIRTPRTPARVTGGVFLVDKNPHNTTESRLVVDFSQFSRGNTRVSWPKFAVPNLQSLTNLLSSNLSWLSLDVSAAFYHLPLHPAAMPHLLVGSSGLSRYVARLSSNSRIINNQHRTMQNLHDSCSRNLYVSLMLLYKTYGRKLHLYSHPIILGFRKIPMGVGLSPFLLAQFTSAICSVVRRAFPHCLAFSYMHDVVLGAKSVQHLESLYAAVTNFLLSLGIHLNPHKTKRWGYSLNFMGYVIGSWGTLPQEHIVQKIKMCFRKLPVNRPIDWKVCQRIVGLLGFAAPFTQCGYPALMPLYACIQAKQAFTFSPTYKAFLSKQYLHLYPVARQRPGLCQVFADATPTGWGLAIGHQRMRGAFVSPLPIHTAHLLAACFARSRSGAKLIGTDNSVVLSRKYTSFPWLLGCAANWILRGTSFVYVPSALNPADDPSRGRLGLYRPLLRLLYRPTTGRTSLYADSPSVPSHLPDRVHFASPLHVAWRPP

SEQ ID NO: 17 - protein, 1026 aa, Artificial Sequence
  source: /note="Description of Artificial Sequence: Synthetic polypeptide"
MDIDPYKEFGASVELLSFLPSDFFPSVRDLLDTASALYREALESPEHCSPHHTALRQAILCWGELMNLATWVGSNLEDPASRELVVSYVNVNMGLKIRQLLWFHISCLTFGRETVLEYLVSFGVWIRTPPAYRPPNAPILSTLPETTVVRRRGRSPRRRTPSPRRRRSQSPRRRRSQSRESQCMPLSYQHFRKLLLLDDEAGPLEEELPRLADEDLNRRVAEDLNLGNLNVSIPWTHKVGNFTGLYSSTVPVFNPEWQTPSFPHIHLQEDIINRCQQYVGPLTVNEKRRLKLIMPARFYPNLTKYLPLDKGIKPYYPEHTVNHYFKTRHYLHTLWKAGILYKRETTRSASFCGSPYSWEQELQHGRLVFQTSTRHGDESFCSQSSGILSRSPVGPCIRSQLKQSRLGLQPQQGSLARSKSGRSGSIRARVHPTTRQSFGVEPSGSGHIDNSASSASSCLHQSAVRKTAYSHLSTSKRQSSSGHAVELHNFPPSSARSQSEGPLLSCWWLQFRNSKPCSDYCLSHIVNLLEDWGPCTEHGEHNIRIPRTPARVTGGVFLVDKNPHNTTESRLVVDFSQFSRGSTHVSWPKFAVPNLQSLTNLLSSNLSWLSLDVSAAFYHLPLHPAAMPHLLVGSSGLSRYVARLSSTSRNINYQHGAMQDLHDSCSRNLYVSLLLLYKTFGRKLHLYSHPIILGFRKIPMGVGLSPFLLAQFTSAICSVVRRAFPHCLAFSYMHDVVLGAKSVQHLESLFTAVTNFLLSLGIHLNPNKTKRWGYSLNFMGYVIGSWGTLPQEHIVLKIKQCFRKLPVNRPIDWKVCQRIVGLLGFAAPFTQCGYPALMPLYACIQAKQAFTFSPTYKAFLCKQYLNLYPVARQRSGLCQVFADATPTGWGLAVGHQRMRGTFVSPLPIHTAHLLAACFARSRSGAKLIGTDNSVVLSRKYTSFPWLLGCAANWILRGTSFVYVPSALNPADDPSRGRLGLYRPLLRLPFRPTTGRTSLYAVSPSVPSHLPVRVHFASPLHVAWRPP

SEQ ID NO: 18 - protein, 1015 aa, Artificial Sequence
  source: /note="Description of Artificial Sequence: Synthetic polypeptide"
MDIDPYKEFGASVELLSFLPSDFFPSVRDLLDTASALYREALESPEHCSPHHTALRQAILCWGELMNLATWVGVNLEDPASRDLVVSYVNTNMGLKFRQLLWFHISCLTFGRETVLEYLVSFGVWIRTPPAYRPPNAPILSTLPETTVVRRRGRSPRRRTPSPRRRRSQSPRRRRSQSRESQCMPLSYQHFRRLLLLDDEAGPLEEELPRLADEGLNRRVAEDLNLGNLNVSIPWTHKVGNFTGLYSSTVPVFNPHWKTPSFPNIHLHQDIIKKCEQFVGPLTVNEKRRLQLIMPARFYPNVTKYLPLDKGIKPYYPEHLVNHYFQTRHYLHTLWKAGILYKRETTHSASFCGSPYSWEQELQHGAESFHQQSSGILSRPPVGSSLQSKHRKSRLGLQSQQGHLARRQQGRGWSIRAGIHPTARRPFGVEPSGSGHTANLASKSASCLYQSAVRKAAYPVVSTFKKHSSSGHAVELHNLPPNSARSQSERPVFPCWWLQFRNSKPCSDYCLSHIVNLLEDWGPCAEHGEHHIRIPRTPARVTGGVFLVDKNPHNTAESRLVVDFSQFSRGNYRVSWPKFAVPNLQSLTNLLSSNLSWLSLDVSAAFYHLPLHPAAMPHLLVGSSGLSRYVARLSSNSRIFNYQHGTMQNLHDSCSRNLYVSLMLLYQTFGRKLHLYSHPIILGFRKIPMGVGLSPFLLAQFTSAICSVVRRAFPHCLAFSYMHDVVLGAKSVQHLESLFTAVTNFLLSLGIHLNPNKTKRWGYSLHFMGYVIGCYGSLPQDHIIQKIKECFRKLPVNRPIDWKVCQRIVGLLGFAAPFTQCGYPALMPLYACIQSKQAFTFSPTYKAFLCKQYLNLYPVARQRPGLCQVFADATPTGWGLVMGHQRMRGTFKAPLPIHTAHLLAACFARSRSGANILGTDNSVVLSRKYTSFPWLLGCAANWILRGTSFVYVPSALNPADDPSRGRLGLYRPLLRLPFRPTTGRTSLYADSPSVPSHLPDRVHFASPLHVAWRPP

SEQ ID NO: 19 - protein, 940 aa, Artificial Sequence
  source: /note="Description of Artificial Sequence: Synthetic polypeptide"
MDIDPYKEFGASVELLSFLPSDFFPSVRDLLDTASALYREALESPEHCSPHHTALRQAILCWGELMTLATWVGNNLEDPASRDLVVNYVNTNMGLKIRQLLWFHISCLTFGRETVLEYLVSFGVWIRTPPAYRPPNAPILSTLPETTVVRRRDRGRSPRRRTPSPRRRRSQSPRRRRSQSRESQCMPLSYQHFRKLLLLDDETEAGPLEEELPRLADEDLNRRVAEDLNLGNLNVSIPWTHKVGNFTGLYSSTVPIFNPEWQTPSFPKIHLHEDIANRCQQFVGPLTVNEKRRLRLIMPARFYPNSTKYLPLDKGIKPYYPDHVVNHYFQTRHYLHTLWKAGILYKRETTRSASFCGSPYSWEQELHHGRLVIKTSQRHGDEPFCSQPSGILSRSSVGPEFHSFPPSSARSQSQGPVFSCWWLQFRNTQPCSKYCLSHLVNLLEDWGPCDEHGEHHIRIPRTPARVTGGVFLVDKNPHNTAESRLVVDFSQFSRGITRVSWPKFAVPNLQSLTNLLSSNLSWLSLDVSAAFYHIPLHPAAMPHLLVGSSGLSRYVARLSSNSRIHNNQHGTLQNLHDSCSRQLYVSLMLLYKTYGRKLHLYSHPIILGFRKIPMGVGLSPFLLAQFTSAICSVVRRAFPHCLAFSYMHDVVLGAKSVQHLESLYTAVTNFLLSLGIHLNPNKTKRWGYSLNFMGYVIGSWGTLPQDHIVQKIKHCFRKLPINRPIDWKVCQRIVGLLGFAAPFTQCGYPALMPLYACIQAKQAFTFSPTYKAFLSKQYLNLYPVARQRPGLCQVFADATPTGWGLAIGHQRMRGTFVAPLPIHTAHLLAACFARSRSGAKLIGTDNSVVLSRKYTSFPWLLGCTANWILRGTSFVYVPSALNPADDPSRGRLGLYRPLLRLPYRPTTGRTSLYAVSPSVPSHLPVRVHFASPLHVAWRPP

SEQ ID NO: 20 - protein, 932 aa, Artificial Sequence
  source: /note="Description of Artificial Sequence: Synthetic polypeptide"
MDIDPYKEFGASVELLSFLPSDFFPSVRDLLDTASALYREALESPEHCSPHHTALRQAILCWGELMNLATWVGSNLEDPASRELVVSYVNVNMGLKIRQLLWFHISCLTFGRETVLEYLVSFGVWIRTPPAYRPPNAPILSTLPETTVVRRRGRSPRRRTPSPRRRRSQSPRRRRSQSRESQCMPLSYQHFRKLLLLDDEAGPLEEELPRLADEGLNRRVAEDLNLGNLNVSIPWTHKVGNFTGLYSSTVPVFNPEWQTPSFPHIHLQEDIINRCQQYVGPLTVNEKRRLKLIMPARFYPNLTKYLPLDKGIKPYYPEHVVNHYFQTRHYLHTLWKAGILYKRESTRSASFCGSPYSWEQDLQHGRLVFQTSKRHGDKSFCPQSPGILPRSELHHFPPSSSRSQSQGPVLSCWWLQFRNSEPCSEYCLCHIVNLIEDWGPCTEHGEHRIRTPRTPARVTGGVFLVDKNPHNTTESRLVVDFSQFSRGNTRVSWPKFAVPNLQSLTNLLSSNLSWLSLDVSAAFYHLPLHPAAMPHLLVGSSGLSRYVARLSSNSRIINNQHRTMQNLHDSCSRNLYVSLMLLYKTYGRKLHLYSHPIILGFRKIPMGVGLSPFLLAQFTSAICSVVRRAFPHCLAFSYMHDVVLGAKSVQHLESLYAAVTNFLLSLGIHLNPHKTKRWGYSLNFMGYVIGSWGTLPQEHIVQKIKMCFRKLPVNRPIDWKVCQRIVGLLGFAAPFTQCGYPALMPLYACIQAKQAFTFSPTYKAFLSKQYLHLYPVARQRPGLCQVFADATPTGWGLAIGHQRMRGAFVSPLPIHTAHLLAACFARSRSGAKLIGTDNSVVLSRKYTSFPWLLGCAANWILRGTSFVYVPSALNPADDPSRGRLGLYRPLLRLLYRPTTGRTSLYADSPSVPSHLPDRVHFASPLHVAWRPP

SEQ ID NO: 21 - protein, 936 aa, Artificial Sequence
  source: /note="Description of Artificial Sequence: Synthetic polypeptide"
MDIDPYKEFGASVELLSFLPSDFFPSVRDLLDTASALYREALESPEHCSPHHTALRQAILCWGELMNLATWVGSNLEDPASRELVVSYVNVNMGLKIRQLLWFHISCLTFGRETVLEYLVSFGVWIRTPPAYRPPNAPILSTLPETTVVRRRGRSPRRRTPSPRRRRSQSPRRRRSQSRESQCMPLSYQHFRKLLLLDDEAGPLEEELPRLADEDLNRRVAEDLNLGNLNVSIPWTHKVGNFTGLYSSTVPVFNPEWQTPSFPHIHLQEDIINRCQQYVGPLTVNEKRRLKLIMPARFYPNLTKYLPLDKGIKPYYPEHTVNHYFKTRHYLHTLWKAGILYKRETTRSASFCGSPYSWEQELQHGRLVFQTSTRHGDESFCSQSSGILSRSPVGPELHNFPPSSARSQSEGPLLSCWWLQFRNSKPCSDYCLSHIVNLLEDWGPCTEHGEHNIRIPRTPARVTGGVFLVDKNPHNTTESRLVVDFSQFSRGSTHVSWPKFAVPNLQSLTNLLSSNLSWLSLDVSAAFYHLPLHPAAMPHLLVGSSGLSRYVARLSSTSRNINYQHGAMQDLHDSCSRNLYVSLLLLYKTFGRKLHLYSHPIILGFRKIPMGVGLSPFLLAQFTSAICSVVRRAFPHCLAFSYMHDVVLGAKSVQHLESLFTAVTNFLLSLGIHLNPNKTKRWGYSLNFMGYVIGSWGTLPQEHIVLKIKQCFRKLPVNRPIDWKVCQRIVGLLGFAAPFTQCGYPALMPLYACIQAKQAFTFSPTYKAFLCKQYLNLYPVARQRSGLCQVFADATPTGWGLAVGHQRMRGTFVSPLPIHTAHLLAACFARSRSGAKLIGTDNSVVLSRKYTSFPWLLGCAANWILRGTSFVYVPSALNPADDPSRGRLGLYRPLLRLPFRPTTGRTSLYAVSPSVPSHLPVRVHFASPLHVAWRPP

SEQ ID NO: 22 - protein, 925 aa, Artificial Sequence
  source: /note="Description of Artificial Sequence: Synthetic polypeptide"
MDIDPYKEFGASVELLSFLPSDFFPSVRDLLDTASALYREALESPEHCSPHHTALRQAILCWGELMNLATWVGVNLEDPASRDLVVSYVNTNMGLKFRQLLWFHISCLTFGRETVLEYLVSFGVWIRTPPAYRPPNAPILSTLPETTVVRRRGRSPRRRTPSPRRRRSQSPRRRRSQSRESQCMPLSYQHFRRLLLLDDEAGPLEEELPRLADEGLNRRVAEDLNLGNLNVSIPWTHKVGNFTGLYSSTVPVFNPHWKTPSFPNIHLHQDIIKKCEQFVGPLTVNEKRRLQLIMPARFYPNVTKYLPLDKGIKPYYPEHLVNHYFQTRHYLHTLWKAGILYKRETTHSASFCGSPYSWEQELQHGAESFHQQSSGILSRPPVGSELHNLPPNSARSQSERPVFPCWWLQFRNSKPCSDYCLSHIVNLLEDWGPCAEHGEHHIRIPRTPARVTGGVFLVDKNPHNTAESRLVVDFSQFSRGNYRVSWPKFAVPNLQSLTNLLSSNLSWLSLDVSAAFYHLPLHPAAMPHLLVGSSGLSRYVARLSSNSRIFNYQHGTMQNLHDSCSRNLYVSLMLLYQTFGRKLHLYSHPIILGFRKIPMGVGLSPFLLAQFTSAICSVVRRAFPHCLAFSYMHDVVLGAKSVQHLESLFTAVTNFLLSLGIHLNPNKTKRWGYSLHFMGYVIGCYGSLPQDHIIQKIKECFRKLPVNRPIDWKVCQRIVGLLGFAAPFTQCGYPALMPLYACIQSKQAFTFSPTYKAFLCKQYLNLYPVARQRPGLCQVFADATPTGWGLVMGHQRMRGTFKAPLPIHTAHLLAACFARSRSGANILGTDNSVVLSRKYTSFPWLLGCAANWILRGTSFVYVPSALNPADDPSRGRLGLYRPLLRLPFRPTTGRTSLYADSPSVPSHLPDRVHFASPLHVAWRPP

SEQ ID NO: 23 - protein, 890 aa, Artificial Sequence
  source: /note="Description of Artificial Sequence: Synthetic polypeptide"
MDIDPYKEFGASVELLSFLPSDFFPSVRDLLDTASALYREALESPEHCSPHHTALRQAILCWGELMTLATWVGNNLEDPASRDLVVNYVNTNMGLKIRQLLWFHISCLTFGRETVLEYLVSFGVWIRTPPAYRPPNAPILSTLPETTVVRRRDRGRSPRRRTPSPRRRRSQSPRRRRSQSRESQCMPLSYQHFRKLLLLDDETEAGPLEEELPRLADEDLNRRVAEDLNLGNLNVSIPWTHKVGNFTGLYSSTVPIFNPEWQTPSFPKIHLHEDIANRCQQFVGPLTVNEKRRLRLIMPARFYPNSTKYLPLDKGIKPYYPDHVVNHYFQTRHYLHTLWKAGILYKRETTRSASFCGSPYSWEQELHHGCWWLQFRNTQPCSKYCLSHLVNLLEDWGPCDEHGEHHIRIPRTPARVTGGVFLVDKNPHNTAESRLVVDFSQFSRGITRVSWPKFAVPNLQSLTNLLSSNLSWLSLDVSAAFYHIPLHPAAMPHLLVGSSGLSRYVARLSSNSRIHNNQHGTLQNLHDSCSRQLYVSLMLLYKTYGRKLHLYSHPIILGFRKIPMGVGLSPFLLAQFTSAICSVVRRAFPHCLAFSYMHDVVLGAKSVQHLESLYTAVTNFLLSLGIHLNPNKTKRWGYSLNFMGYVIGSWGTLPQDHIVQKIKHCFRKLPINRPIDWKVCQRIVGLLGFAAPFTQCGYPALMPLYACIQAKQAFTFSPTYKAFLSKQYLNLYPVARQRPGLCQVFADATPTGWGLAIGHQRMRGTFVAPLPIHTAHLLAACFARSRSGAKLIGTDNSVVLSRKYTSFPWLLGCTANWILRGTSFVYVPSALNPADDPSRGRLGLYRPLLRLPYRPTTGRTSLYAVSPSVPSHLPVRVHFASPLHVAWRPP

SEQ ID NO: 24 - protein, 886 aa, Artificial Sequence
  source: /note="Description of Artificial Sequence: Synthetic polypeptide"
MDIDPYKEFGASVELLSFLPSDFFPSVRDLLDTASALYREALESPEHCSPHHTALRQAILCWGELMNLATWVGSNLEDPASRELVVSYVNVNMGLKIRQLLWFHISCLTFGRETVLEYLVSFGVWIRTPPAYRPPNAPILSTLPETTVVRRRGRSPRRRTPSPRRRRSQSPRRRRSQSRESQCMPLSYQHFRKLLLLDDEAGPLEEELPRLADEGLNRRVAEDLNLGNLNVSIPWTHKVGNFTGLYSSTVPVFNPEWQTPSFPHIHLQEDIINRCQQYVGPLTVNEKRRLKLIMPARFYPNLTKYLPLDKGIKPYYPEHVVNHYFQTRHYLHTLWKAGILYKRESTRSASFCGSPYSWEQDLQHGCWWLQFRNSEPCSEYCLCHIVNLIEDWGPCTEHGEHRIRTPRTPARVTGGVFLVDKNPHNTTESRLVVDFSQFSRGNTRVSWPKFAVPNLQSLTNLLSSNLSWLSLDVSAAFYHLPLHPAAMPHLLVGSSGLSRYVARLSSNSRIINNQHRTMQNLHDSCSRNLYVSLMLLYKTYGRKLHLYSHPIILGFRKIPMGVGLSPFLLAQFTSAICSVVRRAFPHCLAFSYMHDVVLGAKSVQHLESLYAAVTNFLLSLGIHLNPHKTKRWGYSLNFMGYVIGSWGTLPQEHIVQKIKMCFRKLPVNRPIDWKVCQRIVGLLGFAAPFTQCGYPALMPLYACIQAKQAFTFSPTYKAFLSKQYLHLYPVARQRPGLCQVFADATPTGWGLAIGHQRMRGAFVSPLPIHTAHLLAACFARSRSGAKLIGTDNSVVLSRKYTSFPWLLGCAANWILRGTSFVYVPSALNPADDPSRGRLGLYRPLLRLLYRPTTGRTSLYADSPSVPSHLPDRVHFASPLHVAWRPP

SEQ ID NO: 25 - protein, 886 aa, Artificial Sequence
  source: /note="Description of Artificial Sequence: Synthetic polypeptide"
MDIDPYKEFGASVELLSFLPSDFFPSVRDLLDTASALYREALESPEHCSPHHTALRQAILCWGELMNLATWVGSNLEDPASRELVVSYVNVNMGLKIRQLLWFHISCLTFGRETVLEYLVSFGVWIRTPPAYRPPNAPILSTLPETTVVRRRGRSPRRRTPSPRRRRSQSPRRRRSQSRESQCMPLSYQHFRKLLLLDDEAGPLEEELPRLADEDLNRRVAEDLNLGNLNVSIPWTHKVGNFTGLYSSTVPVFNPEWQTPSFPHIHLQEDIINRCQQYVGPLTVNEKRRLKLIMPARFYPNLTKYLPLDKGIKPYYPEHTVNHYFKTRHYLHTLWKAGILYKRETTRSASFCGSPYSWEQELQHGCWWLQFRNSKPCSDYCLSHIVNLLEDWGPCTEHGEHNIRIPRTPARVTGGVFLVDKNPHNTTESRLVVDFSQFSRGSTHVSWPKFAVPNLQSLTNLLSSNLSWLSLDVSAAFYHLPLHPAAMPHLLVGSSGLSRYVARLSSTSRNINYQHGAMQDLHDSCSRNLYVSLLLLYKTFGRKLHLYSHPIILGFRKIPMGVGLSPFLLAQFTSAICSVVRRAFPHCLAFSYMHDVVLGAKSVQHLESLFTAVTNFLLSLGIHLNPNKTKRWGYSLNFMGYVIGSWGTLPQEHIVLKIKQCFRKLPVNRPIDWKVCQRIVGLLGFAAPFTQCGYPALMPLYACIQAKQAFTFSPTYKAFLCKQYLNLYPVARQRSGLCQVFADATPTGWGLAVGHQRMRGTFVSPLPIHTAHLLAACFARSRSGAKLIGTDNSVVLSRKYTSFPWLLGCAANWILRGTSFVYVPSALNPADDPSRGRLGLYRPLLRLPFRPTTGRTSLYAVSPSVPSHLPVRVHFASPLHVAWRPP

SEQ ID NO: 26 - protein, 886 aa, Artificial Sequence
  source: /note="Description of Artificial Sequence: Synthetic polypeptide"
MDIDPYKEFGASVELLSFLPSDFFPSVRDLLDTASALYREALESPEHCSPHHTALRQAILCWGELMNLATWVGVNLEDPASRDLVVSYVNTNMGLKFRQLLWFHISCLTFGRETVLEYLVSFGVWIRTPPAYRPPNAPILSTLPETTVVRRRGRSPRRRTPSPRRRRSQSPRRRRSQSRESQCMPLSYQHFRRLLLLDDEAGPLEEELPRLADEGLNRRVAEDLNLGNLNVSIPWTHKVGNFTGLYSSTVPVFNPHWKTPSFPNIHLHQDIIKKCEQFVGPLTVNEKRRLQLIMPARFYPNVTKYLPLDKGIKPYYPEHLVNHYFQTRHYLHTLWKAGILYKRETTHSASFCGSPYSWEQELQHGCWWLQFRNSKPCSDYCLSHIVNLLEDWGPCAEHGEHHIRIPRTPARVTGGVFLVDKNPHNTAESRLVVDFSQFSRGNYRVSWPKFAVPNLQSLTNLLSSNLSWLSLDVSAAFYHLPLHPAAMPHLLVGSSGLSRYVARLSSNSRIFNYQHGTMQNLHDSCSRNLYVSLMLLYQTFGRKLHLYSHPIILGFRKIPMGVGLSPFLLAQFTSAICSVVRRAFPHCLAFSYMHDVVLGAKSVQHLESLFTAVTNFLLSLGIHLNPNKTKRWGYSLHFMGYVIGCYGSLPQDHIIQKIKECFRKLPVNRPIDWKVCQRIVGLLGFAAPFTQCGYPALMPLYACIQSKQAFTFSPTYKAFLCKQYLNLYPVARQRPGLCQVFADATPTGWGLVMGHQRMRGTFKAPLPIHTAHLLAACFARSRSGANILGTDNSVVLSRKYTSFPWLLGCAANWILRGTSFVYVPSALNPADDPSRGRLGLYRPLLRLPFRPTTGRTSLYADSPSVPSHLPDRVHFASPLHVAWRPP

SEQ ID NO: 27 - DNA, 2247 bp, Artificial Sequence
  source: /note="Description of Artificial Sequence: Synthetic polynucleotide"
atgcccctgagctaccagcacttcaggaagctgctgctgctggatgatgaggctggccctctggaggaggagctgcccaggctggcagatgagggcctcaacaggagagtggcagaggacctgaacctgggcaacctgaatgtgagcatcccctggacccacaaagtggggaacttcactggcctctacagcagcacagtgccagtgttcaaccctgagtggcagaccccctccttcccccacatccacctccaggaggacatcatcaacagatgtcagcagtatgtgggccctctgacagtcaatgagaagaggaggctgaagctgatcatgcctgccaggttctaccccaacctgaccaagtacctcccactggacaagggcatcaagccatactatcctgagcatgtggtgaaccactactttcagaccaggcactacctgcacacactgtggaaggctggcatcctgtacaagagggagagcaccagatcagcctctttctgtggctccccctacagctgggagcaggatctccagcatggcagactggtgttccagacctccaagaggcatggggacaagtccttttgcccccagagccctggcatcctgcccaggagcgagctccaccacttccccccctcctccagcagaagccagtcccagggacctgtgctgtcctgctggtggctccagttcaggaacagtgagccctgcagtgagtactgtctgtgtcacattgtgaacctgattgaggactgggggccctgcactgagcatggagagcacaggatcagaacccccaggaccccagccagagtgactggaggtgtgttcctggtggacaagaacccccacaacaccacagagagcagactggtggtggacttctcccagttttcaaggggcaacaccagagtgtcctggcccaagtttgcagtgcccaacctccagagcctgaccaacctgctgtcatcaaacctgagctggctgtccctggatgtgtctgctgccttctaccacctgcccctgcaccctgcagccatgcctcacctcctggtgggcagctcaggcctgagcaggtatgtggccaggctgtcaagcaactccagaatcatcaacaaccagcacaggaccatgcagaacctgcatgactcttgcagcaggaacctgtatgtgagcctgatgctgctgtacaagacctatggcaggaagctgcacctgtactcccaccccatcatcctgggtttcaggaagatccccatgggagtgggactgtcccccttcctgctggcccagttcacctctgccatctgctctgtggtgaggagagccttcccccactgcctggccttctcctacatgcatgatgtggtgctgggggccaagtcagtgcagcacctggagtctctgtatgctgcagtcaccaacttcctgctcagcctgggcatccacctgaacccccacaagaccaagaggtggggctactctctgaacttcatgggctatgtgataggcagctggggcaccctgccacaggagcacatagtgcagaagatcaagatgtgcttcaggaagctgccagtgaacaggcccattgattggaaggtgtgccagaggattgtgggcctgctgggctttgcagcacccttcacacagtgtggctacccagctctgatgcccctgtatgcctgcatccaggccaagcaggccttcaccttctcccccacttacaaggccttcctgtccaagcagtacctgcacctgtaccctgtggcaaggcagaggccaggcctctgccaggtgtttgcagatgccacccccacaggctggggcctggccattggccaccagaggatgagaggggcctttgtgagcccactgccaatccacacagcccacctgctggcagcatgctttgccaggtccaggtctggtgcaaagctgattggcactgacaacagtgtggtgctgtccagaaagtacaccagcttcccctggctgctgggatgtgctgccaactggattctgaggggcaccagctttgtctatgtgccctctgcactgaaccctgcagatgacccctccaggggcagactggggctgtacaggccactgctcagactgctgtacaggcccaccactggcagaacctccctgtatgcagacagcccctcagtgccctctcacctgccagacagagtgcactttgccagccccctgcatgttgcctggaggcccccc

SEQ ID NO: 28 - DNA, 2109 bp, Artificial Sequence
  source: /note="Description of Artificial Sequence: Synthetic polynucleotide"
atgcccctgagctaccagcacttcaggaagctgctgctgctggatgatgaggctggccctctggaggaggagctgcccaggctggcagatgagggcctcaacaggagagtggcagaggacctgaacctgggcaacctgaatgtgagcatcccctggacccacaaagtggggaacttcactggcctctacagcagcacagtgccagtgttcaaccctgagtggcagaccccctccttcccccacatccacctccaggaggacatcatcaacagatgtcagcagtatgtgggccctctgacagtcaatgagaagaggaggctgaagctgatcatgcctgccaggttctaccccaacctgaccaagtacctcccactggacaagggcatcaagccatactatcctgagcatgtggtgaaccactactttcagaccaggcactacctgcacacactgtggaaggctggcatcctgtacaagagggagagcaccagatcagcctctttctgtggctccccctacagctgggagcaggatctccagcatggctgctggtggctccagttcaggaacagtgagccctgcagtgagtactgtctgtgtcacattgtgaacctgattgaggactgggggccctgcactgagcatggagagcacaggatcagaacccccaggaccccagccagagtgactggaggtgtgttcctggtggacaagaacccccacaacaccacagagagcagactggtggtggacttctcccagttttcaaggggcaacaccagagtgtcctggcccaagtttgcagtgcccaacctccagagcctgaccaacctgctgtcatcaaacctgagctggctgtccctggatgtgtctgctgccttctaccacctgcccctgcaccctgcagccatgcctcacctcctggtgggcagctcaggcctgagcaggtatgtggccaggctgtcaagcaactccagaatcatcaacaaccagcacaggaccatgcagaacctgcatgactcttgcagcaggaacctgtatgtgagcctgatgctgctgtacaagacctatggcaggaagctgcacctgtactcccaccccatcatcctgggtttcaggaagatccccatgggagtgggactgtcccccttcctgctggcccagttcacctctgccatctgctctgtggtgaggagagccttcccccactgcctggccttctcctacatgcatgatgtggtgctgggggccaagtcagtgcagcacctggagtctctgtatgctgcagtcaccaacttcctgctcagcctgggcatccacctgaacccccacaagaccaagaggtggggctactctctgaacttcatgggctatgtgataggcagctggggcaccctgccacaggagcacatagtgcagaagatcaagatgtgcttcaggaagctgccagtgaacaggcccattgattggaaggtgtgccagaggattgtgggcctgctgggctttgcagcacccttcacacagtgtggctacccagctctgatgcccctgtatgcctgcatccaggccaagcaggccttcaccttctcccccacttacaaggccttcctgtccaagcagtacctgcacctgtaccctgtggcaaggcagaggccaggcctctgccaggtgtttgcagatgccacccccacaggctggggcctggccattggccaccagaggatgagaggggcctttgtgagcccactgccaatccacacagcccacctgctggcagcatgctttgccaggtccaggtctggtgcaaagctgattggcactgacaacagtgtggtgctgtccagaaagtacaccagcttcccctggctgctgggatgtgctgccaactggattctgaggggcaccagctttgtctatgtgccctctgcactgaaccctgcagatgacccctccaggggcagactggggctgtacaggccactgctcagactgctgtacaggcccaccactggcagaacctccctgtatgcagacagcccctcagtgccctctcacctgccagacagagtgcactttgccagccccctgcatgttgcctggaggcccccc

SEQ ID NO: 29 - DNA, 1602 bp, Artificial Sequence
  source: /note="Description of Artificial Sequence: Synthetic polynucleotide"
atgtccagcagaagccagtcccagggacctgtgctgtcctgctggtggctccagttcaggaacagtgagccctgcagtgagtactgtctgtgtcacattgtgaacctgattgaggactgggggccctgcactgagcatggagagcacaggatcagaacccccaggaccccagccagagtgactggaggtgtgttcctggtggacaagaacccccacaacaccacagagagcagactggtggtggacttctcccagttttcaaggggcaacaccagagtgtcctggcccaagtttgcagtgcccaacctccagagcctgaccaacctgctgtcatcaaacctgagctggctgtccctggatgtgtctgctgccttctaccacctgcccctgcaccctgcagccatgcctcacctcctggtgggcagctcaggcctgagcaggtatgtggccaggctgtcaagcaactccagaatcatcaacaaccagcacaggaccatgcagaacctgcatgactcttgcagcaggaacctgtatgtgagcctgatgctgctgtacaagacctatggcaggaagctgcacctgtactcccaccccatcatcctgggtttcaggaagatccccatgggagtgggactgtcccccttcctgctggcccagttcacctctgccatctgctctgtggtgaggagagccttcccccactgcctggccttctcctacatgcatgatgtggtgctgggggccaagtcagtgcagcacctggagtctctgtatgctgcagtcaccaacttcctgctcagcctgggcatccacctgaacccccacaagaccaagaggtggggctactctctgaacttcatgggctatgtgataggcagctggggcaccctgccacaggagcacatagtgcagaagatcaagatgtgcttcaggaagctgccagtgaacaggcccattgattggaaggtgtgccagaggattgtgggcctgctgggctttgcagcacccttcacacagtgtggctacccagctctgatgcccctgtatgcctgcatccaggccaagcaggccttcaccttctcccccacttacaaggccttcctgtccaagcagtacctgcacctgtaccctgtggcaaggcagaggccaggcctctgccaggtgtttgcagatgccacccccacaggctggggcctggccattggccaccagaggatgagaggggcctttgtgagcccactgccaatccacacagcccacctgctggcagcatgctttgccaggtccaggtctggtgcaaagctgattggcactgacaacagtgtggtgctgtccagaaagtacaccagcttcccctggctgctgggatgtgctgccaactggattctgaggggcaccagctttgtctatgtgccctctgcactgaaccctgcagatgacccctccaggggcagactggggctgtacaggccactgctcagactgctgtacaggcccaccactggcagaacctccctgtatgcagacagcccctcagtgccctctcacctgccagacagagtgcactttgccagccccctgcatgttgcctggaggcccccc

SEQ ID NO: 30 - DNA, 2226 bp, Artificial Sequence
  source: /note="Description of Artificial Sequence: Synthetic polynucleotide"
atgcccctgagctaccaacacttcaggagactgctgctgctggatgatgaggcaggccctctggaggaggagctgcccaggctggcagatgagggcctgaacaggagggtggctgaggacctgaacctgggcaacctgaatgtgagcatcccttggacccacaaagtgggcaacttcacaggcctgtacagcagcactgtgcctgtgttcaacccccactggaagacacccagcttccccaacatccacctgcaccaggacatcatcaagaagtgtgagcagtttgtgggccccctgacagtcaatgagaagaggaggctccagctgatcatgccagccaggttctaccccaatgtgaccaagtacctccccctggacaagggcatcaagccttactatccagagcacctggtgaaccactacttccagaccagacactacctgcacacactgtggaaggcaggcatcctgtacaagagggagaccacacacagtgcctccttctgtggcagcccctactcctgggagcaggagctgcaacatggagctgagtccttccaccagcagtccagtggcatcctgagcaggccccctgtgggcagcgagctgcacaacctgccccccaactctgccagatcccagtctgagaggccagtgttcccttgctggtggctccagttcaggaacagcaagccctgctcagactactgcctgagccacattgtgaacctgctggaggactggggcccctgtgcagagcatggggagcaccacatcagaatccccaggacccctgccagggtgacaggaggggtgttcctggtggacaagaacccccacaacactgcagagtccaggctggtggtggacttctcccagttcagcaggggcaactacagagtctcctggccaaagtttgctgtgcccaacctccagagcctgacaaacctgctgagcagcaacctgtcctggctctccctggatgtgagtgcagccttctatcacctgcccctgcacccagcagccatgccacacctgctggtgggctccagtggcctgtccaggtatgtggccaggctctcctccaactccaggatcttcaactatcagcatggcaccatgcagaacctgcatgacagctgctccaggaacctgtatgtgtccctgatgctgctctatcagacctttggcaggaagctgcacctgtacagccaccccatcatcctggggttcaggaagatccccatgggtgtgggcctgtcccccttcctgctggcccagttcaccagtgccatctgctcagtggtgaggagggccttcccacactgcctggccttctcttacatgcatgatgtggtcctgggtgccaagtctgtgcagcacctggagagcctgttcacagctgtgacaaactttctcctgagcctgggcatccacctgaaccccaacaagaccaagaggtggggttattcactgcacttcatgggctatgtgattggctgctatggctctctgccacaggaccacatcatccagaagatcaaggagtgcttcagaaagctgccagtgaacaggccaattgactggaaggtgtgccagaggattgtgggcctgctgggctttgcagcccccttcacccagtgtggctaccctgccctgatgcccctgtatgcctgcatccagagcaagcaggccttcaccttttcccccacttacaaggccttcctgtgcaagcagtacctgaacctgtaccctgtggccaggcagagacctgggctgtgccaggtgtttgcagatgccacccccacaggatggggactggtcatgggacaccagaggatgaggggcaccttcaaggcacccctgcccatccacacagcccacctgctggctgcctgctttgccaggagcaggagtggggccaacatcctgggcacagacaactctgtggtgctgagcaggaagtacacatccttcccctggctgctgggatgtgcagccaactggatcctgaggggcaccagctttgtgtatgtgccctctgccctcaaccctgcagatgatccaagcaggggcaggctgggactgtacaggccactgctcagactgcccttcaggcccaccactggcaggaccagcctgtatgctgactccccatctgtgccctcccacctgcctgacagagtgcactttgcctccccactgcatgtggcctggaggccccca

SEQ ID NO: 31 - DNA, 2109 bp, Artificial Sequence
  source: /note="Description of Artificial Sequence: Synthetic polynucleotide"
atgcccctgagctaccaacacttcaggagactgctgctgctggatgatgaggcaggccctctggaggaggagctgcccaggctggcagatgagggcctgaacaggagggtggctgaggacctgaacctgggcaacctgaatgtgagcatcccttggacccacaaagtgggcaacttcacaggcctgtacagcagcactgtgcctgtgttcaacccccactggaagacacccagcttccccaacatccacctgcaccaggacatcatcaagaagtgtgagcagtttgtgggccccctgacagtcaatgagaagaggaggctccagctgatcatgccagccaggttctaccccaatgtgaccaagtacctccccctggacaagggcatcaagccttactatccagagcacctggtgaaccactacttccagaccagacactacctgcacacactgtggaaggcaggcatcctgtacaagagggagaccacacacagtgcctccttctgtggcagcccctactcctgggagcaggagctgcaacatggatgctggtggctccagttcaggaacagcaagccctgctcagactactgcctgagccacattgtgaacctgctggaggactggggcccctgtgcagagcatggggagcaccacatcagaatccccaggacccctgccagggtgacaggaggggtgttcctggtggacaagaacccccacaacactgcagagtccaggctggtggtggacttctcccagttcagcaggggcaactacagagtctcctggccaaagtttgctgtgcccaacctccagagcctgacaaacctgctgagcagcaacctgtcctggctctccctggatgtgagtgcagccttctatcacctgcccctgcacccagcagccatgccacacctgctggtgggctccagtggcctgtccaggtatgtggccaggctctcctccaactccaggatcttcaactatcagcatggcaccatgcagaacctgcatgacagctgctccaggaacctgtatgtgtccctgatgctgctctatcagacctttggcaggaagctgcacctgtacagccaccccatcatcctggggttcaggaagatccccatgggtgtgggcctgtcccccttcctgctggcccagttcaccagtgccatctgctcagtggtgaggagggccttcccacactgcctggccttctcttacatgcatgatgtggtcctgggtgccaagtctgtgcagcacctggagagcctgttcacagctgtgacaaactttctcctgagcctgggcatccacctgaaccccaacaagaccaagaggtggggttattcactgcacttcatgggctatgtgattggctgctatggctctctgccacaggaccacatcatccagaagatcaaggagtgcttcagaaagctgccagtgaacaggccaattgactggaaggtgtgccagaggattgtgggcctgctgggctttgcagcccccttcacccagtgtggctaccctgccctgatgcccctgtatgcctgcatccagagcaagcaggccttcaccttttcccccacttacaaggccttcctgtgcaagcagtacctgaacctgtaccctgtggccaggcagagacctgggctgtgccaggtgtttgcagatgccacccccacaggatggggactggtcatgggacaccagaggatgaggggcaccttcaaggcacccctgcccatccacacagcccacctgctggctgcctgctttgccaggagcaggagtggggccaacatcctgggcacagacaactctgtggtgctgagcaggaagtacacatccttcccctggctgctgggatgtgcagccaactggatcctgaggggcaccagctttgtgtatgtgccctctgccctcaaccctgcagatgatccaagcaggggcaggctgggactgtacaggccactgctcagactgcccttcaggcccaccactggcaggaccagcctgtatgctgactccccatctgtgccctcccacctgcctgacagagtgcactttgcctccccactgcatgtggcctggaggccccca

SEQ ID NO: 32 - DNA, 1602 bp, Artificial Sequence
  source: /note="Description of Artificial Sequence: Synthetic polynucleotide"
atgtctgccagatcccagtctgagaggccagtgttcccttgctggtggctccagttcaggaacagcaagccctgctcagactactgcctgagccacattgtgaacctgctggaggactggggcccctgtgcagagcatggggagcaccacatcagaatccccaggacccctgccagggtgacaggaggggtgttcctggtggacaagaacccccacaacactgcagagtccaggctggtggtggacttctcccagttcagcaggggcaactacagagtctcctggccaaagtttgctgtgcccaacctccagagcctgacaaacctgctgagcagcaacctgtcctggctctccctggatgtgagtgcagccttctatcacctgcccctgcacccagcagccatgccacacctgctggtgggctccagtggcctgtccaggtatgtggccaggctctcctccaactccaggatcttcaactatcagcatggcaccatgcagaacctgcatgacagctgctccaggaacctgtatgtgtccctgatgctgctctatcagacctttggcaggaagctgcacctgtacagccaccccatcatcctggggttcaggaagatccccatgggtgtgggcctgtcccccttcctgctggcccagttcaccagtgccatctgctcagtggtgaggagggccttcccacactgcctggccttctcttacatgcatgatgtggtcctgggtgccaagtctgtgcagcacctggagagcctgttcacagctgtgacaaactttctcctgagcctgggcatccacctgaaccccaacaagaccaagaggtggggttattcactgcacttcatgggctatgtgattggctgctatggctctctgccacaggaccacatcatccagaagatcaaggagtgcttcagaaagctgccagtgaacaggccaattgactggaaggtgtgccagaggattgtgggcctgctgggctttgcagcccccttcacccagtgtggctaccctgccctgatgcccctgtatgcctgcatccagagcaagcaggccttcaccttttcccccacttacaaggccttcctgtgcaagcagtacctgaacctgtaccctgtggccaggcagagacctgggctgtgccaggtgtttgcagatgccacccccacaggatggggactggtcatgggacaccagaggatgaggggcaccttcaaggcacccctgcccatccacacagcccacctgctggctgcctgctttgccaggagcaggagtggggccaacatcctgggcacagacaactctgtggtgctgagcaggaagtacacatccttcccctggctgctgggatgtgcagccaactggatcctgaggggcaccagctttgtgtatgtgccctctgccctcaaccctgcagatgatccaagcaggggcaggctgggactgtacaggccactgctcagactgcccttcaggcccaccactggcaggaccagcctgtatgctgactccccatctgtgccctcccacctgcctgacagagtgcactttgcctccccactgcatgtggcctggaggccccca

SEQ ID NO: 33 - DNA, 1227 bp, Artificial Sequence
  source: /note="Description of Artificial Sequence: Synthetic polynucleotide"
atggacattgacccctacaaggagtttggggccagtgtggagctgctgtcttttctgccatctgacttcttccccagtgtgagggacctgctggacactgcctcagcactgtacagagaggccctggagagcccagagcactgctccccccaccacacagccctgaggcaggccatcctctgctggggggagctgatgaacctggccacctgggtgggctccaacctggaggaccctgcctcaagggagctggtggtcagctatgtcaatgtgaacatgggcctcaagatcaggcagctgctgtggttccacatctcctgcctgacctttggcagggagacagtcctggagtacctggtgagctttggggtgtggatcaggaccccccctgcctacaggccccccaatgctcccatcctgtccaccctgccagagaccactgtggtcaggagaaggggcaggtcccccaggaggagaaccccctctcccaggaggaggagaagccagtcccccaggaggaggaggagccagagcagagagtctcagtgcatggagagcaccacatcaggcttcctgggccccctgctggtgctccaggcaggcttctttctgctgaccaggattctgaccatcccccagtccctggacagctggtggacctccctgaattttctggggggggcccctacctgtcctggccagaactctcagtctcccacctcgaatcactcaccaaccagctgtccccccatctgtcctggctacaggtggatgtgcctgaggagattcatcatcttcctgtgcatcctgctgctgtgcctgatctttctgctggtgctgctggactaccagggcatgctgccagtgtgccctctcatcccaggcagctccaccacatccacaggaccttgcaagacatgcaccacaccagcccagggcaccagcatgttcccctcctgctgttgcaccaagccaacagatggcaactgcacatgcattcccatcccctccagctgggcctttgccaggtttctgtgggagtgggccagtgtgagattttcctggctgtctcttctggtgccctttgtgcagtggtttgtgggcctgtcccctacagtgtggctgagtgtcatctggatgatgtggtactggggcccctccctgtacaacatcctctctccctttctgcctctgctgccaatcttcttttgcctgtgggtgtacatc

SEQ ID NO: 34 - DNA, 1290 bp, Artificial Sequence
  source: /note="Description of Artificial Sequence: Synthetic polynucleotide"
atggacattgacccctacaaggagtttggggccagtgtggagctgctgtcttttctgccatctgacttcttccccagtgtgagggacctgctggacactgcctcagcactgtacagagaggccctggagagcccagagcactgctccccccaccacacagccctgaggcaggccatcctctgctggggggagctgatgaacctggccacctgggtgggctccaacctggaggaccctgcctcaagggagctggtggtcagctatgtcaatgtgaacatgggcctcaagatcaggcagctgctgtggttccacatctcctgcctgacctttggcagggagacagtcctggagtacctggtgagctttggggtgtggatcaggaccccccctgcctacaggccccccaatgctcccatcctgtccaccctgccagagaccactgtggtcaggagaaggggcaggtcccccaggaggagaaccccctctcccaggaggaggagaagccagtcccccaggaggaggaggagccagagcagagagtctcagtgcggcagtggggcaaccaacttcagcctcctgaaacaggcaggggatgtggaggaaaacccaggccccgagagcaccacatcaggcttcctgggccccctgctggtgctccaggcaggcttctttctgctgaccaggattctgaccatcccccagtccctggacagctggtggacctccctgaattttctggggggggcccctacctgtcctggccagaactctcagtctcccacctcgaatcactcaccaaccagctgtccccccatctgtcctggctacaggtggatgtgcctgaggagattcatcatcttcctgtgcatcctgctgctgtgcctgatctttctgctggtgctgctggactaccagggcatgctgccagtgtgccctctcatcccaggcagctccaccacatccacaggaccttgcaagacatgcaccacaccagcccagggcaccagcatgttcccctcctgctgttgcaccaagccaacagatggcaactgcacatgcattcccatcccctccagctgggcctttgccaggtttctgtgggagtgggccagtgtgagattttcctggctgtctcttctggtgccctttgtgcagtggtttgtgggcctgtcccctacagtgtggctgagtgtcatctggatgatgtggtactggggcccctccctgtacaacatcctctctccctttctgcctctgctgccaatcttcttttgcctgtgggtgtacatc

SEQ ID NO: 35 - DNA, 1227 bp, Artificial Sequence
  source: /note="Description of Artificial Sequence: Synthetic polynucleotide"
atggacattgacccctacaaggagtttggggccagtgtggagctgctctccttcctgccctcagacttctttcccagtgtgagggacctgcttgacacagcctctgccctctacagagaggccctggagagcccagagcattgctccccccaccacacagcactgaggcaggccatcctgtgctggggggagctcatgaacctggccacctgggtgggtgtcaacctggaggacccagcttccagggatctggtggtcagctatgtgaacacaaacatgggcctcaagttcaggcagctgctctggttccacatctcctgcctgacctttggcagggagactgtgctggagtacctggtgagctttggagtgtggatcaggaccccacctgcctacaggccccccaatgcccccatcctgtccaccctgcctgagaccacagtggtgaggaggagggggaggtcccccagaaggaggaccccttctcccaggaggaggaggagtcagtctcccaggaggaggaggagccagagcagagagtcccagtgtatggagaacatcacctctggctttctgggacccctgctggtgctccaggcaggctttttcctgctgaccaggatcctgaccatccctcagagcctggactcctggtggacatctctgaattttcttgggggcaccactgtgtgcctgggacagaactcccagtctcccacctccaaccacagcccaacatcctgtccccccatctgcccaggctacaggtggatgtgcctgaggaggttcatcatcttcctgttcatcctgctgctgtgcctgatctttctgctggtgctcctggactatcagggcatgctgccagtgtgcccactgatcccaggcagctccaccacaagcacaggaccttgcaggacatgcaccacacctgcccagggcacttccatgtacccatcttgctgttgcaccaagccatctgatggcaattgcacctgcatccccatcccctcaagctgggcctttggcaagttcctgtgggagtgggcaagtgccagattctcttggctgagcctgctggtcccttttgtgcagtggtttgtgggcctgagccccactgtgtggctgtctgtgatctggatgatgtggtactggggcccctccctgtattcaatcctgagcccttttctgccactgctgcccatcttcttttgtctgtgggtgtacatc

SEQ ID NO: 36 - DNA, 1290 bp, Artificial Sequence
  source: /note="Description of Artificial Sequence: Synthetic polynucleotide"
atggacattgacccctacaaggagtttggggccagtgtggagctgctctccttcctgccctcagacttctttcccagtgtgagggacctgcttgacacagcctctgccctctacagagaggccctggagagcccagagcattgctccccccaccacacagcactgaggcaggccatcctgtgctggggggagctcatgaacctggccacctgggtgggtgtcaacctggaggacccagcttccagggatctggtggtcagctatgtgaacacaaacatgggcctcaagttcaggcagctgctctggttccacatctcctgcctgacctttggcagggagactgtgctggagtacctggtgagctttggagtgtggatcaggaccccacctgcctacaggccccccaatgcccccatcctgtccaccctgcctgagaccacagtggtgaggaggagggggaggtcccccagaaggaggaccccttctcccaggaggaggaggagtcagtctcccaggaggaggaggagccagagcagagagtcccagtgtggcagtggggcaaccaacttcagcctcctgaaacaggcaggggatgtggaggaaaacccaggccccgagaacatcacctctggctttctgggacccctgctggtgctccaggcaggctttttcctgctgaccaggatcctgaccatccctcagagcctggactcctggtggacatctctgaattttcttgggggcaccactgtgtgcctgggacagaactcccagtctcccacctccaaccacagcccaacatcctgtccccccatctgcccaggctacaggtggatgtgcctgaggaggttcatcatcttcctgttcatcctgctgctgtgcctgatctttctgctggtgctcctggactatcagggcatgctgccagtgtgcccactgatcccaggcagctccaccacaagcacaggaccttgcaggacatgcaccacacctgcccagggcacttccatgtacccatcttgctgttgcaccaagccatctgatggcaattgcacctgcatccccatcccctcaagctgggcctttggcaagttcctgtgggagtgggcaagtgccagattctcttggctgagcctgctggtcccttttgtgcagtggtttgtgggcctgagccccactgtgtggctgtctgtgatctggatgatgtggtactggggcccctccctgtattcaatcctgagcccttttctgccactgctgcccatcttcttttgtctgtgggtgtacatc

SEQ ID NO: 37 - DNA, 1290 bp, Artificial Sequence
  source: /note="Description of Artificial Sequence: Synthetic polynucleotide"
atggacattgacccctacaaggagtttggggccagtgtggagctgctgtcttttctgccatctgacttcttccccagtgtgagggacctgctggacactgcctcagcactgtacagagaggccctggagagcccagagcactgctccccccaccacacagccctgaggcaggccatcctctgctggggggagctgatgaacctggccacctgggtgggcgtcaacctggaggaccctgcctcaagggacctggtggtcagctatgtcaatacgaacatgggcctcaagttcaggcagctgctgtggttccacatctcctgcctgacctttggcagggagacagtcctggagtacctggtgagctttggggtgtggatcaggaccccccctgcctacaggccccccaatgctcccatcctgtccaccctgccagagaccactgtggtcaggagaaggggcaggtcccccaggaggagaaccccctctcccaggaggaggagaagccagtcccccaggaggaggaggagccagagcagagagtctcagtgcggcagtggggcaaccaacttcagcctcctgaaacaggcaggggatgtggaggaaaacccaggccccgagaacatcacatcaggcttcctgggccccctgctggtgctccaggcaggcttctttctgctgaccaggattctgaccatcccccagtccctggacagctggtggacctccctgaattttctgggggggaccactgtctgtcttggccagaactctcagtctcccacctcgaatcactcaccaaccagctgtccccccatctgtcctggctacaggtggatgtgcctgaggagattcatcatcttcctgttcatcctgctgctgtgcctgatctttctgctggtgctgctggactaccagggcatgctgccagtgtgccctctcatcccaggcagctccaccacatccacaggaccttgcaggacatgcaccacaccagcccagggcaccagcatgtacccctcctgctgttgcaccaagccatcagatggcaactgcacatgcattcccatcccctccagctgggcctttggcaagtttctgtgggagtgggccagtgcgagattttcctggctgtctcttctggtgccctttgtgcagtggtttgtgggcctgtcccctacagtgtggctgagtgtcatctggatgatgtggtactggggcccctccctgtacagcatcctctctccctttctgcctctgctgccaatcttcttttgcctgtgggtgtacatc

SEQ ID NO: 38 - protein, 409 aa, Artificial Sequence
  source: /note="Description of Artificial Sequence: Synthetic polypeptide"
MDIDPYKEFGASVELLSFLPSDFFPSVRDLLDTASALYREALESPEHCSPHHTALRQAILCWGELMNLATWVGSNLEDPASRELVVSYVNVNMGLKIRQLLWFHISCLTFGRETVLEYLVSFGVWIRTPPAYRPPNAPILSTLPETTVVRRRGRSPRRRTPSPRRRRSQSPRRRRSQSRESQCMESTTSGFLGPLLVLQAGFFLLTRILTIPQSLDSWWTSLNFLGGAPTCPGQNSQSPTSNHSPTSCPPICPGYRWMCLRRFIIFLCILLLCLIFLLVLLDYQGMLPVCPLIPGSSTTSTGPCKTCTTPAQGTSMFPSCCCTKPTDGNCTCIPIPSSWAFARFLWEWASVRFSWLSLLVPFVQWFVGLSPTVWLSVIWMMWYWGPSLYNILSPFLPLLPIFFCLWVYI

SEQ ID NO: 39 - protein, 430 aa, Artificial Sequence
  source: /note="Description of Artificial Sequence: Synthetic polypeptide"
MDIDPYKEFGASVELLSFLPSDFFPSVRDLLDTASALYREALESPEHCSPHHTALRQAILCWGELMNLATWVGSNLEDPASRELVVSYVNVNMGLKIRQLLWFHISCLTFGRETVLEYLVSFGVWIRTPPAYRPPNAPILSTLPETTVVRRRGRSPRRRTPSPRRRRSQSPRRRRSQSRESQCGSGATNFSLLKQAGDVEENPGPESTTSGFLGPLLVLQAGFFLLTRILTIPQSLDSWWTSLNFLGGAPTCPGQNSQSPTSNHSPTSCPPICPGYRWMCLRRFIIFLCILLLCLIFLLVLLDYQGMLPVCPLIPGSSTTSTGPCKTCTTPAQGTSMFPSCCCTKPTDGNCTCIPIPSSWAFARFLWEWASVRFSWLSLLVPFVQWFVGLSPTVWLSVIWMMWYWGPSLYNILSPFLPLLPIFFCLWVYI

SEQ ID NO: 40 - protein, 409 aa, Artificial Sequence
  source: /note="Description of Artificial Sequence: Synthetic polypeptide"
MDIDPYKEFGASVELLSFLPSDFFPSVRDLLDTASALYREALESPEHCSPHHTALRQAILCWGELMNLATWVGVNLEDPASRDLVVSYVNTNMGLKFRQLLWFHISCLTFGRETVLEYLVSFGVWIRTPPAYRPPNAPILSTLPETTVVRRRGRSPRRRTPSPRRRRSQSPRRRRSQSRESQCMENITSGFLGPLLVLQAGFFLLTRILTIPQSLDSWWTSLNFLGGTTVCLGQNSQSPTSNHSPTSCPPICPGYRWMCLRRFIIFLFILLLCLIFLLVLLDYQGMLPVCPLIPGSSTTSTGPCRTCTTPAQGTSMYPSCCCTKPSDGNCTCIPIPSSWAFGKFLWEWASARFSWLSLLVPFVQWFVGLSPTVWLSVIWMMWYWGPSLYSILSPFLPLLPIFFCLWVYI

SEQ ID NO: 41 - protein, 430 aa, Artificial Sequence
  source: /note="Description of Artificial Sequence: Synthetic polypeptide"
MDIDPYKEFGASVELLSFLPSDFFPSVRDLLDTASALYREALESPEHCSPHHTALRQAILCWGELMNLATWVGVNLEDPASRDLVVSYVNTNMGLKFRQLLWFHISCLTFGRETVLEYLVSFGVWIRTPPAYRPPNAPILSTLPETTVVRRRGRSPRRRTPSPRRRRSQSPRRRRSQSRESQCGSGATNFSLLKQAGDVEENPGPENITSGFLGPLLVLQAGFFLLTRILTIPQSLDSWWTSLNFLGGTTVCLGQNSQSPTSNHSPTSCPPICPGYRWMCLRRFIIFLFILLLCLIFLLVLLDYQGMLPVCPLIPGSSTTSTGPCRTCTTPAQGTSMYPSCCCTKPSDGNCTCIPIPSSWAFGKFLWEWASARFSWLSLLVPFVQWFVGLSPTVWLSVIWMMWYWGPSLYSILSPFLPLLPIFFCLWVYI

SEQ ID NO: 42 - protein, 90 aa, Artificial Sequence
  source: /note="Description of Artificial Sequence: Synthetic polypeptide"
CIRSQFKQSRLGLQPHQGPLATSQSGRSGSIRARVHSPTRRCFGVEPSGSGHIGHSASSSSSCLHQSAVRKAAYSHLSTSKRQSSSGHAV

SEQ ID NO: 43 - protein, 94 aa, Artificial Sequence
  source: /note="Description of Artificial Sequence: Synthetic polypeptide"
SVGPCIQNQLRKSRLGPQPAQGQLAGRQQGGSGSIRARVHPSPWGTVGVEPSGSGHIHNCASNSSSCLHQSAVRKAAYSHISTSKGHSSSGHAV

SEQ ID NO: 44 - protein, 90 aa, Artificial Sequence
  source: /note="Description of Artificial Sequence: Synthetic polypeptide"
CIRSQLKQSRLGLQPQQGSLARSKSGRSGSIRARVHPTTRQSFGVEPSGSGHIDNSASSASSCLHQSAVRKTAYSHLSTSKRQSSSGHAV

SEQ ID NO: 45 - protein, 90 aa, Artificial Sequence
  source: /note="Description of Artificial Sequence: Synthetic polypeptide"
SLQSKHRKSRLGLQSQQGHLARRQQGRGWSIRAGIHPTARRPFGVEPSGSGHTANLASKSASCLYQSAVRKAAYPVVSTFKKHSSSGHAV

SEQ ID NO: 46 - protein, 140 aa, Artificial Sequence
  source: /note="Description of Artificial Sequence: Synthetic polypeptide"
RLVIKTSQRHGDEPFCSQPSGILSRSSVGPCIRSQFKQSRLGLQPHQGPLATSQSGRSGSIRARVHSPTRRCFGVEPSGSGHIGHSASSSSSCLHQSAVRKAAYSHLSTSKRQSSSGHAVEFHSFPPSSARSQSQGPVFS

SEQ ID NO: 47 - protein, 140 aa, Artificial Sequence
  source: /note="Description of Artificial Sequence: Synthetic polypeptide"
RLVFQTSKRHGDKSFCPQSPGILPRSSVGPCIQNQLRKSRLGPQPAQGQLAGRQQGGSGSIRARVHPSPWGTVGVEPSGSGHIHNCASNSSSCLHQSAVRKAAYSHISTSKGHSSSGHAVELHHFPPSSSRSQSQGPVLS

SEQ ID NO: 48 - protein, 140 aa, Artificial Sequence
  source: /note="Description of Artificial Sequence: Synthetic polypeptide"
RLVFQTSTRHGDESFCSQSSGILSRSPVGPCIRSQLKQSRLGLQPQQGSLARSKSGRSGSIRARVHPTTRQSFGVEPSGSGHIDNSASSASSCLHQSAVRKTAYSHLSTSKRQSSSGHAVELHNFPPSSARSQSEGPLLS

SEQ ID NO: 49 - protein, 129 aa, Artificial Sequence
  source: /note="Description of Artificial Sequence: Synthetic polypeptide"
AESFHQQSSGILSRPPVGSSLQSKHRKSRLGLQSQQGHLARRQQGRGWSIRAGIHPTARRPFGVEPSGSGHTANLASKSASCLYQSAVRKAAYPVVSTFKKHSSSGHAVELHNLPPNSARSQSERPVFP

SEQ ID NO: 50 - protein, 309 aa, Artificial Sequence
  source: /note="Description of Artificial Sequence: Synthetic polypeptide"
PLSYQHFRKLLLLDDEAGPLEEELPRLADEGLNRRVAEDLNLGNLNVSIPWTHKVGNFTGLYSSTVPVFNPEWQTPSFPHIHLQEDIINRCQQYVGPLTVNEKRRLKLIMPARFYPNLTKYLPLDKGIKPYYPEHVVNHYFQTRHYLHTLWKAGILYKRESTRSASFCGSPYSWEQDLQHGRLVFQTSKRHGDKSFCPQSPGILPRSSVGPCIQNQLRKSRLGPQPAQGQLAGRQQGGSGSIRARVHPSPWGTVGVEPSGSGHIHNCASNSSSCLHQSAVRKAAYSHISTSKGHSSSGHAVELHHFPPS

SEQ ID NO: 51 - protein, 298 aa, Artificial Sequence
  source: /note="Description of Artificial Sequence: Synthetic polypeptide"
PLSYQHFRRLLLLDDEAGPLEEELPRLADEGLNRRVAEDLNLGNLNVSIPWTHKVGNFTGLYSSTVPVFNPHWKTPSFPNIHLHQDIIKKCEQFVGPLTVNEKRRLQLIMPARFYPNVTKYLPLDKGIKPYYPEHLVNHYFQTRHYLHTLWKAGILYKRETTHSASFCGSPYSWEQELQHGAESFHQQSSGILSRPPVGSSLQSKHRKSRLGLQSQQGHLARRQQGRGWSIRAGIHPTARRPFGVEPSGSGHTANLASKSASCLYQSAVRKAAYPVVSTFKKHSSSGHAVELHNLPPN

SEQ ID NO: 52 - protein, 845 aa, Artificial Sequence
  source: /note="Description of Artificial Sequence: Synthetic polypeptide"
MPLSYQHFRKLLLLDDETEAGPLEEELPRLADEDLNRRVAEDLNLGNLNVSIPWTHKVGNFTGLYSSTVPIFNPEWQTPSFPKIHLHEDIANRCQQFVGPLTVNEKRRLRLIMPARFYPNSTKYLPLDKGIKPYYPDHVVNHYFQTRHYLHTLWKAGILYKRETTRSASFCGSPYSWEQELHHGRLVIKTSQRHGDEPFCSQPSGILSRSSVGPCIRSQFKQSRLGLQPHQGPLATSQSGRSGSIRARVHSPTRRCFGVEPSGSGHIGHSASSSSSCLHQSAVRKAAYSHLSTSKRQSSSGHAVEFHSFPPSSARSQSQGPVFSCWWLQFRNTQPCSKYCLSHLVNLLEDWGPCDEHGEHHIRIPRTPARVTGGVFLVDKNPHNTAESRLVVDFSQFSRGITRVSWPKFAVPNLQSLTNLLSSNLSWLSLDVSAAFYHIPLHPAAMPHLLVGSSGLSRYVARLSSNSRIHNNQHGTLQNLHDSCSRQLYVSLMLLYKTYGRKLHLYSHPIILGFRKIPMGVGLSPFLLAQFTSAICSVVRRAFPHCLAFSYMHDVVLGAKSVQHLESLYTAVTNFLLSLGIHLNPNKTKRWGYSLNFMGYVIGSWGTLPQDHIVQKIKHCFRKLPINRPIDWKVCQRIVGLLGFAAPFTQCGYPALMPLYACIQAKQAFTFSPTYKAFLSKQYLNLYPVARQRPGLCQVFADATPTGWGLAIGHQRMRGTFVAPLPIHTAHLLAACFARSRSGAKLIGTDNSVVLSRKYTSFPWLLGCTANWILRGTSFVYVPSALNPADDPSRGRLGLYRPLLRLPYRPTTGRTSLYAVSPSVPSHLPVRVHFASPLHVAWRPP

SEQ ID NO: 53 - protein, 843 aa, Artificial Sequence
  source: /note="Description of Artificial Sequence: Synthetic polypeptide"
MPLSYQHFRKLLLLDDEAGPLEEELPRLADEGLNRRVAEDLNLGNLNVSIPWTHKVGNFTGLYSSTVPVFNPEWQTPSFPHIHLQEDIINRCQQYVGPLTVNEKRRLKLIMPARFYPNLTKYLPLDKGIKPYYPEHVVNHYFQTRHYLHTLWKAGILYKRESTRSASFCGSPYSWEQDLQHGRLVFQTSKRHGDKSFCPQSPGILPRSSVGPCIQNQLRKSRLGPQPAQGQLAGRQQGGSGSIRARVHPSPWGTVGVEPSGSGHIHNCASNSSSCLHQSAVRKAAYSHISTSKGHSSSGHAVELHHFPPSSSRSQSQGPVLSCWWLQFRNSEPCSEYCLCHIVNLIEDWGPCTEHGEHRIRTPRTPARVTGGVFLVDKNPHNTTESRLVVDFSQFSRGNTRVSWPKFAVPNLQSLTNLLSSNLSWLSLDVSAAFYHLPLHPAAMPHLLVGSSGLSRYVARLSSNSRIINNQHRTMQNLHDSCSRNLYVSLMLLYKTYGRKLHLYSHPIILGFRKIPMGVGLSPFLLAQFTSAICSVVRRAFPHCLAFSYMHDVVLGAKSVQHLESLYAAVTNFLLSLGIHLNPHKTKRWGYSLNFMGYVIGSWGTLPQEHIVQKIKMCFRKLPVNRPIDWKVCQRIVGLLGFAAPFTQCGYPALMPLYACIQAKQAFTFSPTYKAFLSKQYLHLYPVARQRPGLCQVFADATPTGWGLAIGHQRMRGAFVSPLPIHTAHLLAACFARSRSGAKLIGTDNSVVLSRKYTSFPWLLGCAANWILRGTSFVYVPSALNPADDPSRGRLGLYRPLLRLLYRPTTGRTSLYADSPSVPSHLPDRVHFASPLHVAWRPP

SEQ ID NO: 54 - protein, 843 aa, Artificial Sequence
  source: /note="Description of Artificial Sequence: Synthetic polypeptide"
MPLSYQHFRKLLLLDDEAGPLEEELPRLADEDLNRRVAEDLNLGNLNVSIPWTHKVGNFTGLYSSTVPVFNPEWQTPSFPHIHLQEDIINRCQQYVGPLTVNEKRRLKLIMPARFYPNLTKYLPLDKGIKPYYPEHTVNHYFKTRHYLHTLWKAGILYKRETTRSASFCGSPYSWEQELQHGRLVFQTSTRHGDESFCSQSSGILSRSPVGPCIRSQLKQSRLGLQPQQGSLARSKSGRSGSIRARVHPTTRQSFGVEPSGSGHIDNSASSASSCLHQSAVRKTAYSHLSTSKRQSSSGHAVELHNFPPSSARSQSEGPLLSCWWLQFRNSKPCSDYCLSHIVNLLEDWGPCTEHGEHNIRIPRTPARVTGGVFLVDKNPHNTTESRLVVDFSQFSRGSTHVSWPKFAVPNLQSLTNLLSSNLSWLSLDVSAAFYHLPLHPAAMPHLLVGSSGLSRYVARLSSTSRNINYQHGAMQDLHDSCSRNLYVSLLLLYKTFGRKLHLYSHPIILGFRKIPMGVGLSPFLLAQFTSAICSVVRRAFPHCLAFSYMHDVVLGAKSVQHLESLFTAVTNFLLSLGIHLNPNKTKRWGYSLNFMGYVIGSWGTLPQEHIVLKIKQCFRKLPVNRPIDWKVCQRIVGLLGFAAPFTQCGYPALMPLYACIQAKQAFTFSPTYKAFLCKQYLNLYPVARQRSGLCQVFADATPTGWGLAVGHQRMRGTFVSPLPIHTAHLLAACFARSRSGAKLIGTDNSVVLSRKYTSFPWLLGCAANWILRGTSFVYVPSALNPADDPSRGRLGLYRPLLRLPFRPTTGRTSLYAVSPSVPSHLPVRVHFASPLHVAWRPP

SEQ ID NO: 55 - protein, 832 aa, Artificial Sequence
  source: /note="Description of Artificial Sequence: Synthetic polypeptide"
MPLSYQHFRRLLLLDDEAGPLEEELPRLADEGLNRRVAEDLNLGNLNVSIPWTHKVGNFTGLYSSTVPVFNPHWKTPSFPNIHLHQDIIKKCEQFVGPLTVNEKRRLQLIMPARFYPNVTKYLPLDKGIKPYYPEHLVNHYFQTRHYLHTLWKAGILYKRETTHSASFCGSPYSWEQELQHGAESFHQQSSGILSRPPVGSSLQSKHRKSRLGLQSQQGHLARRQQGRGWSIRAGIHPTARRPFGVEPSGSGHTANLASKSASCLYQSAVRKAAYPVVSTFKKHSSSGHAVELHNLPPNSARSQSERPVFPCWWLQFRNSKPCSDYCLSHIVNLLEDWGPCAEHGEHHIRIPRTPARVTGGVFLVDKNPHNTAESRLVVDFSQFSRGNYRVSWPKFAVPNLQSLTNLLSSNLSWLSLDVSAAFYHLPLHPAAMPHLLVGSSGLSRYVARLSSNSRIFNYQHGTMQNLHDSCSRNLYVSLMLLYQTFGRKLHLYSHPIILGFRKIPMGVGLSPFLLAQFTSAICSVVRRAFPHCLAFSYMHDVVLGAKSVQHLESLFTAVTNFLLSLGIHLNPNKTKRWGYSLHFMGYVIGCYGSLPQDHIIQKIKECFRKLPVNRPIDWKVCQRIVGLLGFAAPFTQCGYPALMPLYACIQSKQAFTFSPTYKAFLCKQYLNLYPVARQRPGLCQVFADATPTGWGLVMGHQRMRGTFKAPLPIHTAHLLAACFARSRSGANILGTDNSVVLSRKYTSFPWLLGCAANWILRGTSFVYVPSALNPADDPSRGRLGLYRPLLRLPFRPTTGRTSLYADSPSVPSHLPDRVHFASPLHVAWRPP

SEQ ID NO: 56 - protein, 19 aa, Artificial Sequence
  source: /note="Description of Artificial Sequence: Synthetic peptide"
ATNFSLLKQAGDVEENPGP

SEQ ID NO: 57 - protein, 24 aa, Artificial Sequence
  source: /note="Description of Artificial Sequence: Synthetic peptide"
APVKQTLNFDLLKLAGDVESNPGP

SEQ ID NO: 58 - protein, 20 aa, Artificial Sequence
  source: /note="Description of Artificial Sequence: Synthetic peptide"
QCTNYALLKLAGDVESNPGP

SEQ ID NO: 59 - protein, 18 aa, Artificial Sequence
  source: /note="Description of Artificial Sequence: Synthetic peptide"
EGRGSLLTCGDVEENPGP

SEQ ID NO: 60 - protein, 4 aa, Unknown
  source: /note="Description of Unknown: furin recognition/cleavage site"
RAKR

SEQ ID NO: 61 - protein, 4 aa, Unknown
  source: /note="Description of Unknown: furin recognition/cleavage site"
REKR

SEQ ID NO: 62 - protein, 4 aa, Unknown
  source: /note="Description of Unknown: furin recognition/cleavage site"
RRKR

SEQ ID NO: 63 - protein, 4 aa, Artificial Sequence
  source: /note="Description of Artificial Sequence: Synthetic peptide"
GGGS

SEQ ID NO: 64 - protein, 185 aa, Hepatitis B virus
MDIDPYKEFGASVELLSFLPSDFFPSVRDLLDTASALYREALESPEHCSPHHTALRQAILCWGELMTLATWVGNNLEDPASRDLVVNYVNTNMGLKIRQLLWFHISCLTFGRETVLEYLVSFGVWIRTPPAYRPPNAPILSTLPETTVVRRRDRGRSPRRRTPSPRRRRSQSPRRRRSQSRESQC

SEQ ID NO: 65 - protein, 183 aa, Hepatitis B virus
MDIDPYKEFGASVELLSFLPSDFFPSVRDLLDTASALYREALESPEHCSPHHTALRQAILCWGELMNLATWVGSNLEDPASRELVVSYVNVNMGLKIRQLLWFHISCLTFGRETVLEYLVSFGVWIRTPPAYRPPNAPILSTLPETTVVRRRGRSPRRRTPSPRRRRSQSPRRRRSQSRESQC

SEQ ID NO: 66 - protein, 183 aa, Hepatitis B virus
MDIDPYKEFGASVELLSFLPSDFFPSVRDLLDTASALYREALESPEHCSPHHTALRQAILCWGELMNLATWVGVNLEDPASRDLVVSYVNTNMGLKFRQLLWFHISCLTFGRETVLEYLVSFGVWIRTPPAYRPPNAPILSTLPETTVVRRRGRSPRRRTPSPRRRRSQSPRRRRSQSRESQC

SEQ ID NO: 67 - protein, 18 aa, Unknown
  source: /note="Description of Unknown: CSF2, GM-CSF sequence"
MWLQSLLLLGTVACSISV

SEQ ID NO: 68 - protein, 23 aa, Unknown
  source: /note="Description of Unknown: PLAT, t-PA sequence"
MDAMKRGLCCVLLLCGAVFVSAR

SEQ ID NO: 69 - protein, 16 aa, Unknown
  source: /note="Description of Unknown: CD74 sequence"
MHRRRSRSCREDQKPV

SEQ ID NO: 70 - protein, 17 aa, Unknown
  source: /note="Description of Unknown: serum albumin sequence"
KWVTFISLLFLFSSAYS

SEQ ID NO: 71 - protein, 31 aa, Unknown
  source: /note="Description of Unknown: beta-catenin sequence"
MRKAAVSHWQQQSYLDSGIHSGATTTAPSLS

SEQ ID NO: 72 - protein, 107 aa, Unknown
  source: /note="Description of Unknown: CCL7, MCP-3 sequence"
MNPSAAVIFCLILLGLSGTQGILDMAQPVGINTSTTCCYRFINKKIPKQRLESYRRTTSSHCPREAVIFKTKLDKEICADPTQKWVQDFMKHLDKKTQTPKLASAGA

SEQ ID NO: 73 - protein, 76 aa, Unknown [sequence omitted]

SEQ ID NO: 74 - protein, 17 aa, Unknown
  source: /note="Description of Unknown: calreticulin sequence"
MLLSVPLLLGLLGLAVA

SEQ ID NO: 75 - protein, 16 aa, Vesicular stomatitis virus
MKCLLYLAFLFIGVNC

SEQ ID NO: 76 - protein, 21 aa, Unknown
  source: /note="Description of Unknown: CXCL10, IP-10 sequence"
MNQTAILICCLIFLTLSGIQG

SEQ ID NO: 77 - protein, 384 aa, Unknown
  source: /note="Description of Unknown: LAMP-1, N-terminal sequence"
MAPRSARRPLLLLLLLLLLGLMHCASAAMFMVKNGNGTACIMANFSAAFSVNYDTKSGPKNMTLDLPSDATVVLNRSSCGKENTSDPSLVIAFGRGHTLTLNFTRNATRYSVQLMSFVYNLSDTHLFPNASSKEIKTVESITDIRADIDKKYRCVSGTQVHMNNVTVTLHDATIQAYLSNSSFSRGETRCEQDRPSPTTAPPAPPSPSPSPVPKSPSVDKYNVSGTNGTCLLASMGLQLNLTYERKDNTTVTRLLNINPNKTSASGSCGAHLVTLELHSEGTTVLLFQFGMNASSSRFFLQGIQLNTLLPDARDPAFKAANGSLRALQATVGNSYKCNAEEHVRVTKAFSVNIFKVWVQAFKVEGGQFGSVEECLLDENSLEDI

SEQ ID NO: 78 - protein, 39 aa, Unknown
  source: /note="Description of Unknown: LAMP-1, C-terminal sequence"
GSEFTLIPIAVGGALAGLVIVLIAYLVGRKRSHAGYQTI

SEQ ID NO: 79 - protein, 55 aa, Artificial Sequence
  source: /note="Description of Artificial Sequence: Synthetic polypeptide"
  VARIANT (7)..(7): /replace="T"
  VARIANT (11)..(11): /replace="A"
  VARIANT (19)..(19): /replace="G"
  VARIANT (24)..(24): /replace="G"
  VARIANT (29)..(29): /replace="S"
  VARIANT (31)..(31): /replace="T"
  VARIANT (32)..(32): /replace="I"
  VARIANT (36)..(36): /replace="P"
  VARIANT (39)..(39): /replace="V"
  VARIANT (41)..(41): /replace="H"
  VARIANT (42)..(42): /replace="I"
  VARIANT (47)..(47): /replace="A"
  VARIANT (53)..(53): /replace="V"
  VARIANT (54)..(54): /replace="M" or "P" or "T"
  SITE (1)..(55): /note="Variant residues given in the sequence have no preference with respect to those in the annotations for variant positions"
MQWNSTAFHQTLQDPRVRALYFPAGGSSLGAVNPVLTTASPLSSIFSRIGDPALN

SEQ ID NO: 80 - protein, 55 aa, Artificial Sequence
  source: /note="Description of Artificial Sequence: Synthetic polypeptide"
MQWNSTAFHQALQDPRVRGLYFPAGGSSSGTVNPAPNIASHISSISARTGDPVTN

SEQ ID NO: 81 - protein, 55 aa, Artificial Sequence
  source: /note="Description of Artificial Sequence: Synthetic polypeptide"
MQWNSTTFHQTLQDPRVRALYFPAGGSSSGTVSPAQNTVSAISSILSKTGDPVPN

SEQ ID NO: 82 - protein, 55 aa, Artificial Sequence
  source: /note="Description of Artificial Sequence: Synthetic polypeptide"
MQWNSTTFHQALLDPRVRGLYFPAGGSSSGTVNPVPTTASPISSIFSRTGDPAPN

SEQ ID NO: 83 - protein, 55 aa, Artificial Sequence
  source: /note="Description of Artificial Sequence: Synthetic polypeptide"
MQWNSTTFHQTLQDPRVRGLYFPAGGSSSGTVNPVPTTASPISSIFSRIGDPALN

SEQ ID NO: 84 - protein, 163 aa, Artificial Sequence
  source: /note="Description of Artificial Sequence: Synthetic polypeptide"
  VARIANT (20)..(20): /replace="A"
  VARIANT (28)..(28): /replace="G" or "R"
  VARIANT (74)..(74): /replace="L"
  VARIANT (77)..(77): /replace="V"
  VARIANT (86)..(86): /replace="A"
  VARIANT (90)..(90): /replace="T"
  VARIANT (103)..(103): /replace="D"
  VARIANT (115)..(115): /replace="T"
  VARIANT (119)..(119): /replace="A"
  VARIANT (127)..(127): /replace="G"
  VARIANT (132)..(132): /replace="G"
  VARIANT (137)..(137): /replace="S"
  VARIANT (139)..(139): /replace="T"
  VARIANT (140)..(140): /replace="I"
  VARIANT (144)..(144): /replace="P"
  VARIANT (147)..(147): /replace="V"
  VARIANT (149)..(149): /replace="H"
  VARIANT (150)..(150): /replace="I"
  VARIANT (155)..(155): /replace="A"
  VARIANT (161)..(161): /replace="V"
  VARIANT (162)..(162): /replace="M" or "P" or "T"
  SITE (1)..(163): /note="Variant residues given in the sequence have no preference with respect to those in the annotations for variant positions"
MGQNLSTSNPLGFFPDHQLDPAFRANTANPDWDFNPNKDTWPDANKVGAGAFGLGFTPPHGGLLGWSPQAQGIIQTLPANPPPASTNRQSGRQPTPLSPPLRNTHPQAMQWNSTAFHQTLQDPRVRALYFPAGGSSLGAVNPVLTTASPLSSIFSRIGDPALN

SEQ ID NO: 85 - protein, 174 aa, Artificial Sequence
  source: /note="Description of Artificial Sequence: Synthetic polypeptide"
MGGWSSKPRKGMGTNLSVPNPLGFFPDHQLDPAFGANSNNPDWDFNPIKDHWPAANQVGVGAFGPGLTPPHGGILGWSPQAQGILTTVSTIPPPASTNRQSGRQPTPISPPLRDSHPQAMQWNSTAFHQALQDPRVRGLYFPAGGSSSGTVNPAPNIASHISSISARTGDPVTN

SEQ ID NO: 86 - protein, 174 aa, Artificial Sequence
  source: /note="Description of Artificial Sequence: Synthetic polypeptide"
MGGWSSKPRKGMGTNLSVPNPLGFFPDHQLDPAFKANSENPDWDLNPHKDNWPDANKVGVGAFGPGFTPPHGGLLGWSPQAQGLLTTVPAAPPPASTNRQSGRQPTPLSPPLRDTHPQAMQWNSTTFHQTLQDPRVRALYFPAGGSSSGTVSPAQNTVSAISSILSKTGDPVPN

SEQ ID NO: 87 - protein, 174 aa, Artificial Sequence
  source: /note="Description of Artificial Sequence: Synthetic polypeptide"
MGGWSSKPRQGMGTNLSVPNPLGFFPDHQLDPAFGANSNNPDWDFNPNKDHWPEANQVGAGAFGPGFTPPHGGLLGWSPQAQGILTTVPAAPPPASTNRQSGRQPTPISPPLRDSHPQAMQWNSTTFHQALLDPRVRGLYFPAGGSSSGTVNPVPTTASPISSIFSRTGDPAPN

SEQ ID NO: 88 - protein, 163 aa, Artificial Sequence
  source: /note="Description of Artificial Sequence: Synthetic polypeptide"
MGQNLSTSNPLGFFPDHQLDPAFRANTANPDWDFNPNKDTWPDANKVGAGAFGLGFTPPHGGLLGWSPQAQGILQTLPANPPPASTNRQSGRQPTPLSPPLRNTHPQAMQWNSTTFHQTLQDPRVRGLYFPAGGSSSGTVNPVPTTASPISSIFSRIGDPALN

SEQ ID NO: 89 - DNA, 1603 bp, Artificial Sequence
  source: /note="Description of Artificial Sequence: Synthetic polynucleotide"
atgtcttcaagatcccagagtcagggccctgtactttcctgctggtggctccagttcaggaacagtgagccctgctccgaatactgtctctgccatatcgtcaatcttatcgaagactggggaccctgtaccgaacatggagaacatcgcatcaggactcctaggacccctgctcgtgttacaggcggggtttttcttgttgacaaaaatcctcacaataccacagagtctagactcgtggtggacttctctcaattttctagggggaacacccgtgtgtcttggccaaaattcgcagtcccaaatctccagtcactcaccaacctgttgtcctccaatttgtcctggttatcgctggatgtgtctgcggcgttttatcatcttcctctgcatcctgctgctatgcctcatcttcttgttggttcttctggactatcaaggtatgttgcccgtttgtcctctaattccaggatcatcaacaaccagcaccggaccatgcaaaacctgcacgactcctgctcaaggaacctctatgtttccctcatgttgctgtacaaaacctacggacggaaactgcacttgtattcccatcccatcatcttgggctttcgcaaaattcctatgggagtgggcctcagtccgtttctcttggctcagtttactagtgccatttgttcagtggttcgtagggctttcccccactgtctggctttcagttatatgcatgatgtggtattgggggccaagtctgtacaacatcttgagtccctttatgccgctgttaccaattttcttttgtctttgggtatacatttaaaccctcacaaaacaaaaagatggggatattcccttaacttcatgggatatgtaattgggagttggggcacattgccgcaggaacatattgtacaaaaaatcaaaatgtgttttaggaaacttcctgtaaaccggcctattgattggaaagtatgtcaacgaattgtgggtcttttggggtttgccgcccctttcacgcaatgtggatatcctgctttaatgcctttatatgcatgtatacaagcaaaacaggcttttactttctcgccaacttacaaggccttcctaagtaaacagtatctgcacctttaccccgttgctcggcaacggcctggtctgtgccaagtgtttgctgacgcaacccccactggttggggcttggccataggccatcagcgcatgcgtggagccttcgtgtctcctctgccgatccatactgcgcatctcctggccgcttgttttgctcgcagcaggtctggggcaaaactcatcgggactgacaattctgtcgtgctctcccgcaagtatacatcctttccatggctgctaggctgtgctgccaactggatcctgcgcgggacgtcctttgtttacgtcccgtcggcgctgaatcccgcggacgacccctcccggggccgcttggggctctaccgcccgcttctccgcttgttgtaccgaccgactacggggcgcacctctctctacgcggactccccgtctgtgccttctcatctgccggaccgtgtgcacttcgcttcacctctgcacgtcgcatggagaccaccgt

SEQ ID NO: 90 - DNA, 1602 bp, Artificial Sequence
  source: /note="Description of Artificial Sequence: Synthetic polynucleotide"
atgtcatccagatcccagagtcagggccctgtcctttcctgttggtggctccagttcaggaacagtgagccctgttctgagtactgtctctgccacattgtcaatctgattgaggactggggcccctgcacagagcatggtgaacacaggatcaggactcccaggacccctgccagggtgactggtggggttttccttgttgacaaaaatcctcacaacaccacagagtcaaggcttgtggtggacttctctcaattttcaagggggaacacaagggtgtcttggcccaaatttgcagtcccaaatctccagtctctgaccaacctgttgtcctccaatttgtcctggttgtctctggatgtctctgctgccttttatcatcttcctctccatcctgctgccatgcctcatcttcttgttggttcttctggcctctctaggtatgttgccagattgtcctccaattccaggatcatcaacaaccagcacaggaccatgcaaaacctgcatgactcctgctccagaaacctctatgtttctctcatgttgctgtacaaaacctatggcaggaaactgcatttgtattcccatcccatcatcttgggcttcaggaaaattcccatgggagtgggcctcagtcccttcctcttggctcagttcaccagtgccatttgttctgttgtcaggagggctttcccccactgtcttgctttcagttacatgcatgatgtggtcttgggggccaagtctgtccaacatcttgagtcactttatgctgctgtgaccaactttcttttgtctttgggcatccatttgaaccctcacaaaaccaaaagatggggctattccctcaatttcatgggctatgtcattgggagttggggcactttgccccaggaacacattgtgcaaaaaatcaagatgtgtttcaggaaacttcctgtgaacaggccaattgactggaaagtctgtcagagaattgtgggtcttttggggtttgcagctcctttcacccaatgtggctatcctgctttgatgcccttgtatgcctgcatccaggccaaacaggctttcactttctcccccacttacaaggccttcctcagcaaacagtatctccacctttaccctgttgcaaggcagaggcctggtctgtgccaagtgtttgctgatgcaacccccactggttggggcttggccattggccatcagagaatgagaggtgcctttgtgtctcctctccccatccacactgctcatctcctggcagcttgctttgcaaggagcaggtctggagccaaactcatagggactgacaattctgtggtgctctccagaaagtacacctcctttccttggctgctgggctgtgcagccaactggatcctgagggggacttcctttgtttatgtcccctctgccctgaatcctgcagatgacccctccaggggcaggttggggctctacagaccccttctcaggttgttgtacagaccaacaacagggaggacctctctctatgcagattccccctctgttccttctcatcttccagacagagtgcactttgcttctcctctgcatgtggcttggagacctccc

SEQ ID NO: 91 - DNA, 1602 bp, Artificial Sequence
  source: /note="Description of Artificial Sequence: Synthetic polynucleotide"
atgtctagcagaagccagtcccagggacctgtgctgtcttgttggtggcttcagtttcggaatagcgagccatgtagcgagtattgcctgtgtcacatcgtgaatctgattgaggattggggaccatgcacagagcacggagagcaccggatcagaacccctaggacaccagcccgcgtgacaggaggcgtgttcctggtggataagaacccccataatacaacagagagcagactggtggtggatttttctcagttttctcggggcaatacaagagtgtcctggccaaagtttgccgtgcccaatctccagagcctgacaaacctgctgtcttctaatctgagctggctgtccctggacgtgtccgccgccttttaccacctgccactgcaccctgccgccatgccccacctgctggtgggcagctccggactgagcagatacgtggcaaggctgtctagcaattctagaattattaataatcagcacagaacaatgcagaatctgcatgattcttgtagcaggaatctgtacgtgagcctgatgctgctgtataagacatatggacgcaagctgcacctgtattctcaccctattattctgggcttccggaagatccctatgggcgtgggactgtccccattcctgctggcccagtttacctccgccatctgctctgtggtgcggagagccttcccacattgtctggccttttcttacatgcacgatgtggtgctgggcgccaaatccgtgcagcacctggagtctctgtatgccgccgtgacaaacttcctgctgagcctgggcatccacctgaatccacataagacaaagcggtggggctattctctgaattttatgggctatgtgatcggcagctggggaaccctgccacaggagcacattgtgcagaagatcaagatgtgctttcgcaagctgcccgtgaatcggcctatcgattggaaggtgtgccagaggatcgtgggactgctgggattcgcagcaccctttacccagtgcggctacccagccctgatgccactgtatgcctgtatccaggccaaacaggccttcaccttttcccctacatataaggcttttctgtctaagcagtacctgcatctgtatccagtggcaaggcagaggccaggactgtgccaggtgtttgcagatgcaacaccaacaggatggggactggcaatcggacaccagaggatgagaggagccttcgtgagcccactgccaattcacaccgcccacctgctggcagcatgctttgcaaggtcccgctctggagcaaagctgattggcaccgataacagcgtggtgctgtccagaaaatacaccagcttcccctggctgctgggatgtgcagcaaattggattctgaggggcaccagcttcgtgtatgtgccttccgccctgaatcctgccgatgatccatctcgaggcagactgggactgtataggccactgctgagactgctgtataggcctaccacaggcagaacatccctgtatgccgacagcccatccgtgccctctcacctgccagatagagtgcatttcgcaagcccactgcatgtggcatggaggccaccc

SEQ ID NO: 92 - DNA, 1602 bp, Artificial Sequence
  source: /note="Description of Artificial Sequence: Synthetic polynucleotide"
atgtcttcaagatcccagagtcagggccctgtactttcctgctggtggctccagttcaggaacagtgagccctgctctgaatactgtctctgccatattgtcaatcttatagaagactggggaccctgtactgaacatggagaacataggatcaggactcctaggacccctgctagagttacagggggggtttttcttgttgacaaaaatcctcacaataccacagagtctagacttgtggtggacttctctcaattttctagggggaacaccagggtgtcttggccaaaatttgcagtcccaaatctccagtcactcaccaacctgttgtcctccaatttgtcctggttatccctggatgtgtctgcagccttttatcatcttcctctgcatcctgctgctatgcctcatcttcttgttggttcttctggactatcaaggtatgttgccaggttgtcctctaattccaggatcatcaacaaccagcacaggaccatgcaaaacctgcatgactcctgctcaaggaacctctatgtttccctcatgttgctgtacaaaacctatggaaggaaactgcacttgtattcccatcccatcatcttgggctttagaaaaattcctatgggagtgggcctcagtccctttctcttggctcagtttactagtgccatttgttcagtggttagaagggctttcccccactgtctggctttcagttatatgcatgatgtggtattgggggccaagtctgtacaacatcttgagtccctttatgctgctgttaccaattttcttttgtctttgggtatacatttaaaccctcacaaaacaaaaagatggggatattcccttaacttcatgggatatgtaattgggagttggggcacattgcctcaggaacatattgtacaaaaaatcaaaatgtgttttaggaaacttcctgtaaacaggcctattgattggaaagtatgtcaaagaattgtgggtcttttggggtttgcagcccctttcacccaatgtggatatcctgctttaatgcctttatatgcatgtatacaagcaaaacaggcttttactttctccccaacttacaaggccttcctaagtaaacagtatctgcacctttaccctgttgctaggcaaaggcctggtctgtgccaagtgtttgctgatgcaacccccactggttggggcttggccataggccatcagaggatgaggggagcctttgtgtctcctctgcctatccatactgcccatctcctggcagcttgttttgctaggagcaggtctggggcaaaactcattgggactgacaattctgttgtgctctccagaaagtatacatcctttccatggctgctaggctgtgctgccaactggatcctgagggggacatcctttgtttatgtcccttcagcactgaatcctgctgatgacccctccaggggcagattggggctctacaggccccttctcaggttgttgtacagacccactactgggagaacctctctctatgcagactccccctctgtgccttctcatctgcctgacagggtgcactttgcttcacctctgcatgttgcatggagaccacct

SEQ ID NO: 93 - DNA, 1602 bp, Artificial Sequence
  source: /note="Description of Artificial Sequence: Synthetic polynucleotide"
atgagttcccgatcacagagtcaggggcccgtcctttcatgttggtggcttcagtttcgaaactccgagccatgttctgagtattgtctctgccacattgtgaatcttattgaagactggggcccctgcaccgagcacggcgagcaccgaatacggacacctcgaacgccagcaagagtgacgggcggagtgttcctcgtcgacaagaatccacacaacacgacggagagtagattggtcgttgatttcagtcaattttcaagaggcaatacacgagtttcttggccgaaattcgccgtaccgaatctgcaatccttgacaaatttgcttagttctaatttgtcttggctttctctcgatgtttccgccgctttctatcacttgccccttcacccagccgcgatgccgcatctcttggtgggcagctctggacttagtagatacgtagctagactcagttctaactcacggataataaataaccaacatcgcactatgcagaacctgcatgattcttgttcccggaacttgtatgtctccttgatgttgttgtataaaacttatgggcgaaagcttcatctgtatagccatccgattatattgggttttaggaaaattcctatgggtgttggcttgagcccttttctgctggcgcaatttacttcagctatctgctcagtagtacgccgggcgtttccccattgtcttgctttctcatacatgcatgatgtagtacttggggccaagtctgtacaacaccttgagagtttgtatgccgccgtaactaatttccttctctctctcgggatccatcttaaccctcacaaaacgaagaggtggggttattctctgaatttcatgggatatgttatcgggtcttggggaacgctgcctcaggaacacatcgtccagaaaatcaagatgtgtttcagaaagttgccagtgaacagaccgatagattggaaggtttgccaaagaattgttggcttgttgggattcgcagccccattcacacagtgcgggtatccggctttgatgcccctttatgcttgtatccaggcaaaacaggcattcaccttttcaccgacttacaaagcatttctttctaagcagtatctccatctttaccctgtcgctcgacagcggccggggctttgccaggttttcgcagacgcaaccccaactggttggggtcttgcgatcggccaccagaggatgcgcggtgcattcgtgtccccgctcccaatccatacggcccacttgctggcggcgtgcttcgctcgaagtagaagcggggctaaattgatcggcacggacaattcagtcgtgttgtcacgcaaatatacctcctttccctggttgctcggttgcgcagcaaactggatacttcggggaactagtttcgtttatgtgccctctgctctcaaccccgccgacgatccttcacgagggaggctgggtctttaccgcccattgctcaggctgctttaccggcctaccactgggagaacaagcttgtacgccgacagcccgagcgtcccgtctcatctgcccgacagagttcactttgcgagtccattgcacgtcgcttggcgcccgccg

SEQ ID NO: 94 - DNA, 1602 bp, Artificial Sequence
  source: /note="Description of Artificial Sequence: Synthetic polynucleotide"
atgagttccagatcacagagtcaggggcctgtcctttcatgttggtggcttcagtttagaaactcagagccatgttctgagtattgtctctgccacattgtgaatcttattgaagactggggcccctgcacagagcatggagagcacagaataaggacacctagaaccccagcaagagtgacaggtggagtgttcctggtagacaagaatccacacaacacaactgagagtagattggtggttgatttcagtcaattttcaagaggcaatacaagagtttcttggccaaaatttgctgtacccaatctgcaatccttgacaaatttgcttagttctaatttgtcttggctttctctagatgtttctgcagctttctatcacttgccccttcacccagcagctatgcctcatctcttggtgggcagctctggacttagtagatatgtagctagactcagttctaactcaaggataataaataaccaacataggactatgcagaacctgcatgattcttgttccaggaacttgtatgtctccttgatgttgttgtataaaacttatgggagaaagcttcatctgtatagccatcctattatattgggttttaggaaaattcctatgggtgttggcttgagcccttttctgctggcccaatttacttcagctatctgctcagtagtaaggagggcctttccccattgtcttgctttctcatacatgcatgatgtagtacttggggccaagtctgtacaacaccttgagagtttgtatgcagcagtaactaatttccttctctctcttgggatccatcttaaccctcacaaaaccaagaggtggggttattctctgaatttcatgggatatgttatagggtcttggggaaccctgcctcaggaacacattgtccagaaaatcaagatgtgtttcagaaagttgccagtgaacagaccaatagattggaaggtttgccaaagaattgttggcttgttgggatttgcagccccattcacacagtgtgggtatcctgctttgatgcccctttatgcttgtatccaggcaaaacaggcattcaccttttcacccacttacaaagcatttctttctaagcagtatctccatctttaccctgtggctagacagaggccagggctttgccaggtttttgcagatgcaaccccaactggttggggtcttgcaattggccaccagaggatgagaggtgcatttgtgtccccactcccaatccatactgcccacttgctggcagcttgctttgctagaagtagaagtggggctaaattgattggcacagacaattcagttgtgttgtcaaggaaatatacctcctttccctggttgcttggttgtgcagcaaactggatacttaggggaactagttttgtttatgtgccctctgctctcaaccctgcagatgatccttcaagagggaggctgggtctttacaggccattgctcaggctgctttacaggcctaccactgggagaacaagcttgtatgcagacagccccagtgtcccctctcatctgcctgacagagttcactttgcaagtccattgcatgttgcttggagacctcca

SEQ ID NO: 95 - protein, 6 aa, Hepatitis B virus
SARSQS

SEQ ID NO: 96 - protein, 6 aa, Hepatitis B virus
SSRSQS

SEQ ID NO: 97 - protein, 4 aa, Hepatitis B virus
YMDD

SEQ ID NO: 98 - protein, 4 aa, Hepatitis B virus
AELL

SEQ ID NO: 99 - protein, 4 aa, Artificial Sequence
  source: /note="Description of Artificial Sequence: Synthetic peptide"
YMHD

SEQ ID NO: 100 - protein, 4 aa, Artificial Sequence
  source: /note="Description of Artificial Sequence: Synthetic peptide"
AHLL

SEQ ID NO: 101 - protein, 8 aa, Hepatitis B virus
MGLKFRQL

SEQ ID NO: 102 - protein, 8 aa, Hepatitis B virus
MGLKIRQL